European Patent Specification EP 2 760 882 B1, published May 24, 2023. Title: Increasing Virus Like Particle Yield in Plants. Applicant: Medicago Inc. The sequence listing filed with the application follows.

SEQUENCE LISTING (64 sequences)

SEQ ID NO: 1 - protein, 5 aa, Artificial Sequence
  proton channel signature sequence
  misc_feature (2)..(4): Xaa can be any naturally occurring amino acid
HXXXW

SEQ ID NO: 2 - DNA, 41 bp, Artificial Sequence
  primer IF-H5A-I-05.s1+3c
aaatttgtcgggcccatggagaaaatagtgcttcttcttgc

SEQ ID NO: 3 - DNA, 50 bp, Artificial Sequence
  primer IF-H5dTm.r
actaaagaaaataggcctttaaatgcaaattctgcattgtaacgatccat

SEQ ID NO: 4 - DNA, 4903 bp, Artificial Sequence
  Construct 1191
tggcaggatatattgtggtgtaaacaaattgacgcttagacaacttaataacacattgcggacgtttttaatgtactgaattaacgccgaatcccgggctggtatatttatatgttgtcaaataactcaaaaaccataaaagtttaagttagcaagtgtgtacatttttacttgaacaaaaatattcacctactactgttataaatcattattaaacattagagtaaagaaatatggatgataagaacaagagtagtgatattttgacaacaattttgttgcaacatttgagaaaattttgttgttctctcttttcattggtcaaaaacaatagagagagaaaaaggaagagggagaataaaaacataatgtgagtatgagagagaaagttgtacaaaagttgtaccaaaatagttgtacaaatatcattgaggaatttgacaaaagctacacaaataagggttaattgctgtaaataaataaggatgacgcattagagagatgtaccattagagaatttttggcaagtcattaaaaagaaagaataaattatttttaaaattaaaagttgagtcatttgattaaacatgtgattatttaatgaattgatgaaagagttggattaaagttgtattagtaattagaatttggtgtcaaatttaatttgacatttgatcttttcctatatattgccccatagagtcagttaactcatttttatatttcatagatcaaataagagaaataacggtatattaatccctccaaaaaaaaaaaacggtatatttactaaaaaatctaagccacgtaggaggataacaggatccccgtaggaggataacatccaatccaaccaatcacaacaatcctgatgagataacccactttaagcccacgcatctgtggcacatctacattatctaaatcacacattcttccacacatctgagccacacaaaaaccaatccacatctttatcacccattctataaaaaatcacactttgtgagtctacactttgattcccttcaaacacatacaaagagaagagactaattaattaattaatcatcttgagagaaaatggaacgagctatacaaggaaacgacgctagggaacaagctaacagtgaacgttgggatggaggatcaggaggtaccacttctcccttcaaacttcctgacgaaagtccgagttggactgagtggcggctacataacgatgagacgaattcgaatcaagataatccccttggtttcaaggaaagctggggtttcgggaaagttgtatttaagagatatctcagatacgacaggacggaagcttcactgcacagagtccttggatcttggacgggagattcggttaactatgcagcatctcgatttttcggtttcgaccagatcggatgtacctatagtattcggtttcgaggagttagtatcaccgtttctggagggtcgcgaactcttcagcatctctgtgagatggcaattcggtctaagcaagaactgctacagcttgccccaatcgaagtggaaagtaatgtatcaagaggatgccctgaaggtactcaaaccttcgaaaaagaaagcgagtaagttaaaatgcttcttcgtctcctatttataatatggtttgttattgttaattttgttcttgtagaagagcttaattaatcgttgttgttatgaaatactatttgtatgagatgaactggtgtaatgtaattcatttacataagtggagtcagaatcagaatgtttcctccataactaactagacatgaagacctgccgcgtacaattgtcttatatttgaacaactaaaattgaacatcttttgccacaactttataagtggttaatatagctcaaatatatggtcaagttcaatagattaataatggaaatatcagttatcgaaattcattaacaatcaacttaacgttattaactactaattttatatcatcccctttgataaatgatagtacaccaattaggaaggagcatgctcgcctaggagattgtcgtttcccgccttcagtttgcaagctgctctagccgtgtagccaatacgcaaaccgcctctccccgcgcgttgggaattactagcgcgtgtcgacaagcttgcatgccggtcaacatggtggagcacgacacacttgtctactccaaaaatatcaaagatacagtctcagaagaccaaagggcaattgagacttttcaacaaagggtaatatccggaaacctcctcggattccattgcccagctatctgtcactttattgtgaagatagtggaaaaggaaggtggctcctacaaatgccatcattgcgataaaggaaaggccatcgttgaagatgcctctgccgacagtggtcccaaagatggacccccacccacgaggagcatcgtggaaaaagaagacgttccaaccacgtcttcaaagcaagtggattgatgtgataacatggtggagcacgacacacttgtctactccaaaaatatcaaagatacagtctcagaagaccaaagggcaattgagacttttcaacaaagggtaatatccggaaacctcctcggattccattgcccagctatctgtcactttattgtgaagatagtggaaaaggaaggtggctcctacaaatgccatcattgcgataaaggaaaggccatcgttgaagatgcctctgccgacagtggtcccaaagatggacccccacccacgaggagcatcgtggaaaaagaagacgttccaaccacgtcttcaaagcaagtggattgatgtgatatctccactgacgtaagggatgacgcacaatcccactatccttcgcaagacccttcctctatataaggaagttcatttcatttggagaggtattaaaatcttaataggttttgataaaagcgaacgtggggaaacccgaaccaaaccttcttctaaactctctctcatctctcttaaagcaaacttctctcttgtctttcttgcgtgagcgatcttcaacgttgtcagatcgtgcttcggcaccagtacaacgttttctttcactgaagcgaaatcaaagatctctttgtggacacgtagtgcggcgccattaaataacgtgtacttgtcctattcttgtcggtgtggtcttgggaaaagaaagcttgctggaggctgctgttcagccccatacattacttgttacgattctgctgactttcggcgggtgcaatatctctacttctgcttgacgaggtattgttgcctgtacttctttcttcttcttcttgctgattggttctataagaaatctagtattttctttgaaacagagttttcccgtggttttcgaacttggagaaagattgttaagcttctgtatattctgcccaaatttgtcgggcccgcggatggcgaaaaacgttgcgattttcggcttattgttttctcttcttgtgttggttccttctcagatcttcgcctgcaggctcctcagccaaaacgacacccccatctgtctatccactggcccctggatctgctgcccaaactaactccatggtgaccctgggatgcctggtcaagggctatttccctgagccagtgacagtgacctggaactctggatccctgtccagcggtgtgcacaccttcccagctgtcctgcagtctgacctctacactctgagcagctcagtgactgtcccctccagcacctggcccagcgagaccgtcacctgcaacgttgcccacccggccagcagcaccaaggtggacaagaaaattgtgcccagggattgtggttgtaagccttgcatatgtacagtcccagaagtatcatctgtcttcatcttccccccaaagcccaaggatgtgctcaccattactctgactcctaaggtcacgtgtgttgtggtagacatcagcaaggatgatcccgaggtccagttcagctggtttgtagatgatgtggaggtgcacacagctcagacgcaaccccgggaggagcagttcaacagcactttccgctcagtcagtgaacttcccatcatgcaccaggactggctcaatggcaaggagcgatcgctcaccatcaccatcaccatcaccatcaccattaaaggcctattttctttagtttgaatttactgttattcggtgtgcatttctatgtttggtgagcggttttctgtgctcagagtgtgtttattttatgtaatttaatttctttgtgagctcctgtttagcaggtcgtcccttcagcaaggacacaaaaagattttaattttattaaaaaaaaaaaaaaaaaagaccgggaattcgatatcaagcttatcgacctgcagatcgttcaaacatttggcaataaagtttcttaagattgaatcctgttgccggtcttgcgatgattatcatataatttctgttgaattacgttaagcatgtaataattaacatgtaatgcatgacgttatttatgagatgggtttttatgattagagtcccgcaattatacatttaatacgcgatagaaaacaaaatatagcgcgcaaactaggataaattatcgcgcgcggtgtcatctatgttactagatctctagagtctcaagcttggcgcgcccacgtgactagtggcactggccgtcgttttacaacgtcgtgactgggaaaaccctggcgttacccaacttaatcgccttgcagcacatccccctttcgccagctggcgtaatagcgaagaggcccgcaccgatcgcccttcccaacagttgcgcagcctgaatggcgaatgctagagcagcttgagcttggatcagattgtcgtttcccgccttcagtttaaactatcagtgtttgacaggatatattggcgggtaaacctaagagaaaagagcgttta

SEQ ID NO: 5 - DNA, 3447 bp, Artificial Sequence
  Expression cassette number 489
gtcaacatggtggagcacgacacacttgtctactccaaaaatatcaaagatacagtctcagaagaccaaagggcaattgagacttttcaacaaagggtaatatccggaaacctcctcggattccattgcccagctatctgtcactttattgtgaagatagtggaaaaggaaggtggctcctacaaatgccatcattgcgataaaggaaaggccatcgttgaagatgcctctgccgacagtggtcccaaagatggacccccacccacgaggagcatcgtggaaaaagaagacgttccaaccacgtcttcaaagcaagtggattgatgtgataacatggtggagcacgacacacttgtctactccaaaaatatcaaagatacagtctcagaagaccaaagggcaattgagacttttcaacaaagggtaatatccggaaacctcctcggattccattgcccagctatctgtcactttattgtgaagatagtggaaaaggaaggtggctcctacaaatgccatcattgcgataaaggaaaggccatcgttgaagatgcctctgccgacagtggtcccaaagatggacccccacccacgaggagcatcgtggaaaaagaagacgttccaaccacgtcttcaaagcaagtggattgatgtgatatctccactgacgtaagggatgacgcacaatcccactatccttcgcaagacccttcctctatataaggaagttcatttcatttggagaggtattaaaatcttaataggttttgataaaagcgaacgtggggaaacccgaaccaaaccttcttctaaactctctctcatctctcttaaagcaaacttctctcttgtctttcttgcgtgagcgatcttcaacgttgtcagatcgtgcttcggcaccagtacaacgttttctttcactgaagcgaaatcaaagatctctttgtggacacgtagtgcggcgccattaaataacgtgtacttgtcctattcttgtcggtgtggtcttgggaaaagaaagcttgctggaggctgctgttcagccccatacattacttgttacgattctgctgactttcggcgggtgcaatatctctacttctgcttgacgaggtattgttgcctgtacttctttcttcttcttcttgctgattggttctataagaaatctagtattttctttgaaacagagttttcccgtggttttcgaacttggagaaagattgttaagcttctgtatattctgcccaaatttgtcgggcccatggagaaaatagtgcttcttcttgcaatagtcagtcttgttaaaagtgatcagatttgcattggttaccatgcaaacaattcaacagagcaggttgacacaatcatggaaaagaacgttactgttacacatgcccaagacatactggaaaagacacacaacgggaagctctgcgatctagatggagtgaagcctctaattttaagagattgtagtgtagctggatggctcctcgggaacccaatgtgtgacgaattcatcaatgtaccggaatggtcttacatagtggagaaggccaatccaaccaatgacctctgttacccagggagtttcaacgactatgaagaactgaaacacctattgagcagaataaaccattttgagaaaattcaaatcatccccaaaagttcttggtccgatcatgaagcctcatcaggagttagctcagcatgtccatacctgggaagtccctccttttttagaaatgtggtatggcttatcaaaaagaacagtacatacccaacaataaagaaaagctacaataataccaaccaagaggatcttttggtactgtggggaattcaccatcctaatgatgcggcagagcagacaaggctatatcaaaacccaaccacctatatttccattgggacatcaacactaaaccagagattggtaccaaaaatagctactagatccaaagtaaacgggcaaagtggaaggatggagttcttctggacaattttaaaacctaatgatgcaatcaacttcgagagtaatggaaatttcattgctccagaatatgcatacaaaattgtcaagaaaggggactcagcaattatgaaaagtgaattggaatatggtaactgcaacaccaagtgtcaaactccaatgggggcgataaactctagtatgccattccacaacatacaccctctcaccatcggggaatgccccaaatatgtgaaatcaaacagattagtccttgcaacagggctcagaaatagccctcaaagagagagcagaagaaaaaagagaggactatttggagctatagcaggttttatagagggaggatggcagggaatggtagatggttggtatgggtaccaccatagcaatgagcaggggagtgggtacgctgcagacaaagaatccactcaaaaggcaatagatggagtcaccaataaggtcaactcaatcattgacaaaatgaacactcagtttgaggccgttggaagggaatttaataacttagaaaggagaatagagaatttaaacaagaagatggaagacgggtttctagatgtctggacttataatgccgaacttctggttctcatggaaaatgagagaactctagactttcatgactcaaatgttaagaacctctacgacaaggtccgactacagcttagggataatgcaaaggagctgggtaacggttgtttcgagttctatcacaaatgtgataatgaatgtatggaaagtataagaaacggaacgtacaactatccgcagtattcagaagaagcaagattaaaaagagaggaaataagtggggtaaaattggaatcaataggaacttaccaaatactgtcaatttattcaacagtggcgagttccctagcactggcaatcatgatggctggtctatctttatggatgtgctccaatggatcgttacaatgcagaatttgcatttaaaggcctattttctttagtttgaatttactgttattcggtgtgcatttctatgtttggtgagcggttttctgtgctcagagtgtgtttattttatgtaatttaatttctttgtgagctcctgtttagcaggtcgtcccttcagcaaggacacaaaaagattttaattttattaaaaaaaaaaaaaaaaaagaccgggaattcgatatcaagcttatcgacctgcagatcgttcaaacatttggcaataaagtttcttaagattgaatcctgttgccggtcttgcgatgattatcatataatttctgttgaattacgttaagcatgtaataattaacatgtaatgcatgacgttatttatgagatgggtttttatgattagagtcccgcaattatacatttaatacgcgatagaaaacaaaatatagcgcgcaaactaggataaattatcgcgcgcggtgtcatctatgttactagat

SEQ ID NO: 6 - protein, 568 aa, Influenza virus
MEKIVLLLAIVSLVKSDQICIGYHANNSTEQVDTIMEKNVTVTHAQDILEKTHNGKLCDLDGVKPLILRDCSVAGWLLGNPMCDEFINVPEWSYIVEKANPTNDLCYPGSFNDYEELKHLLSRINHFEKIQIIPKSSWSDHEASSGVSSACPYLGSPSFFRNVVWLIKKNSTYPTIKKSYNNTNQEDLLVLWGIHHPNDAAEQTRLYQNPTTYISIGTSTLNQRLVPKIATRSKVNGQSGRMEFFWTILKPNDAINFESNGNFIAPEYAYKIVKKGDSAIMKSELEYGNCNTKCQTPMGAINSSMPFHNIHPLTIGECPKYVKSNRLVLATGLRNSPQRESRRKKRGLFGAIAGFIEGGWQGMVDGWYGYHHSNEQGSGYAADKESTQKAIDGVTNKVNSIIDKMNTQFEAVGREFNNLERRIENLNKKMEDGFLDVWTYNAELLVLMENERTLDFHDSNVKNLYDKVRLQLRDNAKELGNGCFEFYHKCDNECMESIRNGTYNYPQYSEEARLKREEISGVKLESIGTYQILSIYSTVASSLALAIMMAGLSLWMCSNGSLQCRICI

SEQ ID NO: 7 - DNA, 42 bp, Artificial Sequence
  primer IF-S1-M1+M2ANC.c
aaatttgtcgggcccatgagtcttctaaccgaggtcgaaacg

SEQ ID NO: 8 - DNA, 43 bp, Artificial Sequence
  primer IF-S1-4-M2ANC.r
actaaagaaaataggcctttactccagctctatgctgacaaaa

SEQ ID NO: 9 - DNA, 294 bp, Artificial Sequence
  nucleotide sequence of synthesized M2 gene (DQ508860)
atgagtcttctaaccgaggtcgaaacgcctatcagaaacgaatgggggtgcagatgcaacgattcaagtgatcctcttgttgttgccgcaagtataattgggattgtgcacctgatattgtggattattgatcgccttttttccaaaagcatttatcgtatctttaaacacggtttaaaaagagggccttctacggaaggagtaccagagtctatgagggaagaatatcgagaggaacagcagaatgctgtggatgctgacgatggtcattttgtcagcatagagctggagtaa

SEQ ID NO: 10 - DNA, 2034 bp, Artificial Sequence
  Expression cassette number 1261
gtcaacatggtggagcacgacacacttgtctactccaaaaatatcaaagatacagtctcagaagaccaaagggcaattgagacttttcaacaaagggtaatatccggaaacctcctcggattccattgcccagctatctgtcactttattgtgaagatagtggaaaaggaaggtggctcctacaaatgccatcattgcgataaaggaaaggccatcgttgaagatgcctctgccgacagtggtcccaaagatggacccccacccacgaggagcatcgtggaaaaagaagacgttccaaccacgtcttcaaagcaagtggattgatgtgataacatggtggagcacgacacacttgtctactccaaaaatatcaaagatacagtctcagaagaccaaagggcaattgagacttttcaacaaagggtaatatccggaaacctcctcggattccattgcccagctatctgtcactttattgtgaagatagtggaaaaggaaggtggctcctacaaatgccatcattgcgataaaggaaaggccatcgttgaagatgcctctgccgacagtggtcccaaagatggacccccacccacgaggagcatcgtggaaaaagaagacgttccaaccacgtcttcaaagcaagtggattgatgtgatatctccactgacgtaagggatgacgcacaatcccactatccttcgcaagacccttcctctatataaggaagttcatttcatttggagaggtattaaaatcttaataggttttgataaaagcgaacgtggggaaacccgaaccaaaccttcttctaaactctctctcatctctcttaaagcaaacttctctcttgtctttcttgcgtgagcgatcttcaacgttgtcagatcgtgcttcggcaccagtacaacgttttctttcactgaagcgaaatcaaagatctctttgtggacacgtagtgcggcgccattaaataacgtgtacttgtcctattcttgtcggtgtggtcttgggaaaagaaagcttgctggaggctgctgttcagccccatacattacttgttacgattctgctgactttcggcgggtgcaatatctctacttctgcttgacgaggtattgttgcctgtacttctttcttcttcttcttgctgattggttctataagaaatctagtattttctttgaaacagagttttcccgtggttttcgaacttggagaaagattgttaagcttctgtatattctgcccaaatttgtcgggcccatgagtcttctaaccgaggtcgaaacgcctatcagaaacgaatgggggtgcagatgcaacgattcaagtgatcctcttgttgttgccgcaagtataattgggattgtgcacctgatattgtggattattgatcgccttttttccaaaagcatttatcgtatctttaaacacggtttaaaaagagggccttctacggaaggagtaccagagtctatgagggaagaatatcgagaggaacagcagaatgctgtggatgctgacgatggtcattttgtcagcatagagctggagtaaaggcctattttctttagtttgaatttactgttattcggtgtgcatttctatgtttggtgagcggttttctgtgctcagagtgtgtttattttatgtaatttaatttctttgtgagctcctgtttagcaggtcgtcccttcagcaaggacacaaaaagattttaattttattaaaaaaaaaaaaaaaaaagaccgggaattcgatatcaagcttatcgacctgcagatcgttcaaacatttggcaataaagtttcttaagattgaatcctgttgccggtcttgcgatgattatcatataatttctgttgaattacgttaagcatgtaataattaacatgtaatgcatgacgttatttatgagatgggtttttatgattagagtcccgcaattatacatttaatacgcgatagaaaacaaaatatagcgcgcaaactaggataaattatcgcgcgcggtgtcatctatgttactagat

SEQ ID NO: 11 - protein, 97 aa, Influenza virus
MSLLTEVETPIRNEWGCRCNDSSDPLVVAASIIGIVHLILWIIDRLFSKSIYRIFKHGLKRGPSTEGVPESMREEYREEQQNAVDADDGHFVSIELE

SEQ ID NO: 12 - DNA, 294 bp, Artificial Sequence
  nucleotide sequence of synthesized M2 gene
atgagtcttctaaccgaggtcgaaacgcctatcagaaacgaatgggggtgcagatgcaacggttcaagtgatcctctcactattgccgcaaatatcattgggatcttgcacttgacattgtggattcttgatcgtctttttttcaaatgcatttaccgtcgctttaaatacggactgaaaggagggccttctacggaaggagtgccaaagtctatgagggaagaatatcgaaaggaacagcagagtgctgtggatgctgacgatggtcattttgtcagcatagagctggagtaa

SEQ ID NO: 13 - DNA, 2034 bp, Artificial Sequence
  Expression cassette number 859
gtcaacatggtggagcacgacacacttgtctactccaaaaatatcaaagatacagtctcagaagaccaaagggcaattgagacttttcaacaaagggtaatatccggaaacctcctcggattccattgcccagctatctgtcactttattgtgaagatagtggaaaaggaaggtggctcctacaaatgccatcattgcgataaaggaaaggccatcgttgaagatgcctctgccgacagtggtcccaaagatggacccccacccacgaggagcatcgtggaaaaagaagacgttccaaccacgtcttcaaagcaagtggattgatgtgataacatggtggagcacgacacacttgtctactccaaaaatatcaaagatacagtctcagaagaccaaagggcaattgagacttttcaacaaagggtaatatccggaaacctcctcggattccattgcccagctatctgtcactttattgtgaagatagtggaaaaggaaggtggctcctacaaatgccatcattgcgataaaggaaaggccatcgttgaagatgcctctgccgacagtggtcccaaagatggacccccacccacgaggagcatcgtggaaaaagaagacgttccaaccacgtcttcaaagcaagtggattgatgtgatatctccactgacgtaagggatgacgcacaatcccactatccttcgcaagacccttcctctatataaggaagttcatttcatttggagaggtattaaaatcttaataggttttgataaaagcgaacgtggggaaacccgaaccaaaccttcttctaaactctctctcatctctcttaaagcaaacttctctcttgtctttcttgcgtgagcgatcttcaacgttgtcagatcgtgcttcggcaccagtacaacgttttctttcactgaagcgaaatcaaagatctctttgtggacacgtagtgcggcgccattaaataacgtgtacttgtcctattcttgtcggtgtggtcttgggaaaagaaagcttgctggaggctgctgttcagccccatacattacttgttacgattctgctgactttcggcgggtgcaatatctctacttctgcttgacgaggtattgttgcctgtacttctttcttcttcttcttgctgattggttctataagaaatctagtattttctttgaaacagagttttcccgtggttttcgaacttggagaaagattgttaagcttctgtatattctgcccaaatttgtcgggcccatgagtcttctaaccgaggtcgaaacgcctatcagaaacgaatgggggtgcagatgcaacggttcaagtgatcctctcactattgccgcaaatatcattgggatcttgcacttgacattgtggattcttgatcgtctttttttcaaatgcatttaccgtcgctttaaatacggactgaaaggagggccttctacggaaggagtgccaaagtctatgagggaagaatatcgaaaggaacagcagagtgctgtggatgctgacgatggtcattttgtcagcatagagctggagtaaaggcctattttctttagtttgaatttactgttattcggtgtgcatttctatgtttggtgagcggttttctgtgctcagagtgtgtttattttatgtaatttaatttctttgtgagctcctgtttagcaggtcgtcccttcagcaaggacacaaaaagattttaattttattaaaaaaaaaaaaaaaaaagaccgggaattcgatatcaagcttatcgacctgcagatcgttcaaacatttggcaataaagtttcttaagattgaatcctgttgccggtcttgcgatgattatcatataatttctgttgaattacgttaagcatgtaataattaacatgtaatgcatgacgttatttatgagatgggtttttatgattagagtcccgcaattatacatttaatacgcgatagaaaacaaaatatagcgcgcaaactaggataaattatcgcgcgcggtgtcatctatgttactagat

SEQ ID NO: 14 - protein, 97 aa, Influenza virus
MSLLTEVETPIRNEWGCRCNGSSDPLTIAANIIGILHLTLWILDRLFFKCIYRRFKYGLKGGPSTEGVPKSMREEYRKEQQSAVDADDGHFVSIELE

SEQ ID NO: 15 - DNA, 46 bp, Artificial Sequence
  primer IF-H1A-C-09.s2+4c
tctcagatcttcgccgacacattatgtataggttatcatgcgaaca

SEQ ID NO: 16 - DNA, 49 bp, Artificial Sequence
  primer IF-H1A-C-09.s1-4r
actaaagaaaataggcctttaaatacatattctacactgtagagaccca

SEQ ID NO: 17 - DNA, 1701 bp, Artificial Sequence
  nucleotide sequence of synthesized H1 gene
atgaaggcaatactagtagttctgctatatacatttgcaaccgcaaatgcagacacattatgtataggttatcatgcgaacaattcaacagacactgtagacacagtactagaaaagaatgtaacagtaacacactctgttaaccttctagaagacaagcataacgggaaactatgcaaactaagaggggtagccccattgcatttgggtaaatgtaacattgctggctggatcctgggaaatccagagtgtgaatcactctccacagcaagctcatggtcctacattgtggaaacacctagttcagacaatggaacgtgttacccaggagatttcatcgattatgaggagctaagagagcaattgagctcagtgtcatcatttgaaaggtttgagatattccccaagacaagttcatggcccaatcatgactcgaacaaaggtgtaacggcagcatgtcctcatgctggagcaaaaagcttctacaaaaatttaatatggctagttaaaaaaggaaattcatacccaaagctcagcaaatcctacattaatgataaagggaaagaagtcctcgtgctatggggcattcaccatccatctactagtgctgaccaacaaagtctctatcagaatgcagatgcatatgtttttgtggggtcatcaagatacagcaagaagttcaagccggaaatagcaataagacccaaagtgagggatcaagaagggagaatgaactattactggacactagtagagccgggagacaaaataacattcgaagcaactggaaatctagtggtaccgagatatgcattcgcaatggaaagaaatgctggatctggtattatcatttcagatacaccagtccacgattgcaatacaacttgtcaaacacccaagggtgctataaacaccagcctcccatttcagaatatacatccgatcacaattggaaaatgtccaaaatatgtaaaaagcacaaaattgagactggccacaggattgaggaatatcccgtctattcaatctagaggcctatttggggccattgccggtttcattgaaggggggtggacagggatggtagatggatggtacggttatcaccatcaaaatgagcaggggtcaggatatgcagccgacctgaagagcacacagaatgccattgacgagattactaacaaagtaaattctgttattgaaaagatgaatacacagttcacagcagtaggtaaagagttcaaccacctggaaaaaagaatagagaatttaaataaaaaagttgatgatggtttcctggacatttggacttacaatgccgaactgttggttctattggaaaatgaaagaactttggactaccacgattcaaatgtgaagaacttatatgaaaaggtaagaagccagctaaaaaacaatgccaaggaaattggaaacggctgctttgaattttaccacaaatgcgataacacgtgcatggaaagtgtcaaaaatgggacttatgactacccaaaatactcagaggaagcaaaattaaacagagaagaaatagatggggtaaagctggaatcaacaaggatttaccagattttggcgatctattcaactgtcgccagttcattggtactggtagtctccctgggggcaatcagtttctggatgtgctctaatgggtctctacagtgtagaatatgtatttaa

SEQ ID NO: 18 - DNA, 4897 bp, Artificial Sequence
  Construct 1192
tggcaggatatattgtggtgtaaacaaattgacgcttagacaacttaataacacattgcggacgtttttaatgtactgaattaacgccgaatcccgggctggtatatttatatgttgtcaaataactcaaaaaccataaaagtttaagttagcaagtgtgtacatttttacttgaacaaaaatattcacctactactgttataaatcattattaaacattagagtaaagaaatatggatgataagaacaagagtagtgatattttgacaacaattttgttgcaacatttgagaaaattttgttgttctctcttttcattggtcaaaaacaatagagagagaaaaaggaagagggagaataaaaacataatgtgagtatgagagagaaagttgtacaaaagttgtaccaaaatagttgtacaaatatcattgaggaatttgacaaaagctacacaaataagggttaattgctgtaaataaataaggatgacgcattagagagatgtaccattagagaatttttggcaagtcattaaaaagaaagaataaattatttttaaaattaaaagttgagtcatttgattaaacatgtgattatttaatgaattgatgaaagagttggattaaagttgtattagtaattagaatttggtgtcaaatttaatttgacatttgatcttttcctatatattgccccatagagtcagttaactcatttttatatttcatagatcaaataagagaaataacggtatattaatccctccaaaaaaaaaaaacggtatatttactaaaaaatctaagccacgtaggaggataacaggatccccgtaggaggataacatccaatccaaccaatcacaacaatcctgatgagataacccactttaagcccacgcatctgtggcacatctacattatctaaatcacacattcttccacacatctgagccacacaaaaaccaatccacatctttatcacccattctataaaaaatcacactttgtgagtctacactttgattcccttcaaacacatacaaagagaagagactaattaattaattaatcatcttgagagaaaatggaacgagctatacaaggaaacgacgctagggaacaagctaacagtgaacgttgggatggaggatcaggaggtaccacttctcccttcaaacttcctgacgaaagtccgagttggactgagtggcggctacataacgatgagacgaattcgaatcaagataatccccttggtttcaaggaaagctggggtttcgggaaagttgtatttaagagatatctcagatacgacaggacggaagcttcactgcacagagtccttggatcttggacgggagattcggttaactatgcagcatctcgatttttcggtttcgaccagatcggatgtacctatagtattcggtttcgaggagttagtatcaccgtttctggagggtcgcgaactcttcagcatctctgtgagatggcaattcggtctaagcaagaactgctacagcttgccccaatcgaagtggaaagtaatgtatcaagaggatgccctgaaggtactcaaaccttcgaaaaagaaagcgagtaagttaaaatgcttcttcgtctcctatttataatatggtttgttattgttaattttgttcttgtagaagagcttaattaatcgttgttgttatgaaatactatttgtatgagatgaactggtgtaatgtaattcatttacataagtggagtcagaatcagaatgtttcctccataactaactagacatgaagacctgccgcgtacaattgtcttatatttgaacaactaaaattgaacatcttttgccacaactttataagtggttaatatagctcaaatatatggtcaagttcaatagattaataatggaaatatcagttatcgaaattcattaacaatcaacttaacgttattaactactaattttatatcatcccctttgataaatgatagtacaccaattaggaaggagcatgctcgcctaggagattgtcgtttcccgccttcagtttgcaagctgctctagccgtgtagccaatacgcaaaccgcctctccccgcgcgttgggaattactagcgcgtgtcgacaagcttgcatgccggtcaacatggtggagcacgacacacttgtctactccaaaaatatcaaagatacagtctcagaagaccaaagggcaattgagacttttcaacaaagggtaatatccggaaacctcctcggattccattgcccagctatctgtcactttattgtgaagatagtggaaaaggaaggtggctcctacaaatgccatcattgcgataaaggaaaggccatcgttgaagatgcctctgccgacagtggtcccaaagatggacccccacccacgaggagcatcgtggaaaaagaagacgttccaaccacgtcttcaaagcaagtggattgatgtgataacatggtggagcacgacacacttgtctactccaaaaatatcaaagatacagtctcagaagaccaaagggcaattgagacttttcaacaaagggtaatatccggaaacctcctcggattccattgcccagctatctgtcactttattgtgaagatagtggaaaaggaaggtggctcctacaaatgccatcattgcgataaaggaaaggccatcgttgaagatgcctctgccgacagtggtcccaaagatggacccccacccacgaggagcatcgtggaaaaagaagacgttccaaccacgtcttcaaagcaagtggattgatgtgatatctccactgacgtaagggatgacgcacaatcccactatccttcgcaagacccttcctctatataaggaagttcatttcatttggagaggtattaaaatcttaataggttttgataaaagcgaacgtggggaaacccgaaccaaaccttcttctaaactctctctcatctctcttaaagcaaacttctctcttgtctttcttgcgtgagcgatcttcaacgttgtcagatcgtgcttcggcaccagtacaacgttttctttcactgaagcgaaatcaaagatctctttgtggacacgtagtgcggcgccattaaataacgtgtacttgtcctattcttgtcggtgtggtcttgggaaaagaaagcttgctggaggctgctgttcagccccatacattacttgttacgattctgctgactttcggcgggtgcaatatctctacttctgcttgacgaggtattgttgcctgtacttctttcttcttcttcttgctgattggttctataagaaatctagtattttctttgaaacagagttttcccgtggttttcgaacttggagaaagattgttaagcttctgtatattctgcccaaatttgtcgggcccatggcgaaaaacgttgcgattttcggcttattgttttctcttcttgtgttggttccttctcagatcttcgccgcggctcctcagccaaaacgacacccccatctgtctatccactggcccctggatctgctgcccaaactaactccatggtgaccctgggatgcctggtcaagggctatttccctgagccagtgacagtgacctggaactctggatccctgtccagcggtgtgcacaccttcccagctgtcctgcagtctgacctctacactctgagcagctcagtgactgtcccctccagcacctggcccagcgagaccgtcacctgcaacgttgcccacccggccagcagcaccaaggtggacaagaaaattgtgcccagggattgtggttgtaagccttgcatatgtacagtcccagaagtatcatctgtcttcatcttccccccaaagcccaaggatgtgctcaccattactctgactcctaaggtcacgtgtgttgtggtagacatcagcaaggatgatcccgaggtccagttcagctggtttgtagatgatgtggaggtgcacacagctcagacgcaaccccgggaggagcagttcaacagcactttccgctcagtcagtgaacttcccatcatgcaccaggactggctcaatggcaaggagcgatcgctcaccatcaccatcaccatcaccatcaccattaaaggcctattttctttagtttgaatttactgttattcggtgtgcatttctatgtttggtgagcggttttctgtgctcagagtgtgtttattttatgtaatttaatttctttgtgagctcctgtttagcaggtcgtcccttcagcaaggacacaaaaagattttaattttattaaaaaaaaaaaaaaaaaagaccgggaattcgatatcaagcttatcgacctgcagatcgttcaaacatttggcaataaagtttcttaagattgaatcctgttgccggtcttgcgatgattatcatataatttctgttgaattacgttaagcatgtaataattaacatgtaatgcatgacgttatttatgagatgggtttttatgattagagtcccgcaattatacatttaatacgcgatagaaaacaaaatatagcgcgcaaactaggataaattatcgcgcgcggtgtcatctatgttactagatctctagagtctcaagcttggcgcgcccacgtgactagtggcactggccgtcgttttacaacgtcgtgactgggaaaaccctggcgttacccaacttaatcgccttgcagcacatccccctttcgccagctggcgtaatagcgaagaggcccgcaccgatcgcccttcccaacagttgcgcagcctgaatggcgaatgctagagcagcttgagcttggatcagattgtcgtttcccgccttcagtttaaactatcagtgtttgacaggatatattggcgggtaaacctaagagaaaagagcgttta

SEQ ID NO: 19 - DNA, 3462 bp, Artificial Sequence
  Expression cassette number 484
gtcaacatggtggagcacgacacacttgtctactccaaaaatatcaaagatacagtctcagaagaccaaagggcaattgagacttttcaacaaagggtaatatccggaaacctcctcggattccattgcccagctatctgtcactttattgtgaagatagtggaaaaggaaggtggctcctacaaatgccatcattgcgataaaggaaaggccatcgttgaagatgcctctgccgacagtggtcccaaagatggacccccacccacgaggagcatcgtggaaaaagaagacgttccaaccacgtcttcaaagcaagtggattgatgtgataacatggtggagcacgacacacttgtctactccaaaaatatcaaagatacagtctcagaagaccaaagggcaattgagacttttcaacaaagggtaatatccggaaacctcctcggattccattgcccagctatctgtcactttattgtgaagatagtggaaaaggaaggtggctcctacaaatgccatcattgcgataaaggaaaggccatcgttgaagatgcctctgccgacagtggtcccaaagatggacccccacccacgaggagcatcgtggaaaaagaagacgttccaaccacgtcttcaaagcaagtggattgatgtgatatctccactgacgtaagggatgacgcacaatcccactatccttcgcaagacccttcctctatataaggaagttcatttcatttggagaggtattaaaatcttaataggttttgataaaagcgaacgtggggaaacccgaaccaaaccttcttctaaactctctctcatctctcttaaagcaaacttctctcttgtctttcttgcgtgagcgatcttcaacgttgtcagatcgtgcttcggcaccagtacaacgttttctttcactgaagcgaaatcaaagatctctttgtggacacgtagtgcggcgccattaaataacgtgtacttgtcctattcttgtcggtgtggtcttgggaaaagaaagcttgctggaggctgctgttcagccccatacattacttgttacgattctgctgactttcggcgggtgcaatatctctacttctgcttgacgaggtattgttgcctgtacttctttcttcttcttcttgctgattggttctataagaaatctagtattttctttgaaacagagttttcccgtggttttcgaacttggagaaagattgttaagcttctgtatattctgcccaaatttgtcgggcccatggcgaaaaacgttgcgattttcggcttattgttttctcttcttgtgttggttccttctcagatcttcgccgacacattatgtataggttatcatgcgaacaattcaacagacactgtagacacagtactagaaaagaatgtaacagtaacacactctgttaaccttctagaagacaagcataacgggaaactatgcaaactaagaggggtagccccattgcatttgggtaaatgtaacattgctggctggatcctgggaaatccagagtgtgaatcactctccacagcaagctcatggtcctacattgtggaaacacctagttcagacaatggaacgtgttacccaggagatttcatcgattatgaggagctaagagagcaattgagctcagtgtcatcatttgaaaggtttgagatattccccaagacaagttcatggcccaatcatgactcgaacaaaggtgtaacggcagcatgtcctcatgctggagcaaaaagcttctacaaaaatttaatatggctagttaaaaaaggaaattcatacccaaagctcagcaaatcctacattaatgataaagggaaagaagtcctcgtgctatggggcattcaccatccatctactagtgctgaccaacaaagtctctatcagaatgcagatgcatatgtttttgtggggtcatcaagatacagcaagaagttcaagccggaaatagcaataagacccaaagtgagggatcaagaagggagaatgaactattactggacactagtagagccgggagacaaaataacattcgaagcaactggaaatctagtggtaccgagatatgcattcgcaatggaaagaaatgctggatctggtattatcatttcagatacaccagtccacgattgcaatacaacttgtcaaacacccaagggtgctataaacaccagcctcccatttcagaatatacatccgatcacaattggaaaatgtccaaaatatgtaaaaagcacaaaattgagactggccacaggattgaggaatatcccgtctattcaatctagaggcctatttggggccattgccggtttcattgaaggggggtggacagggatggtagatggatggtacggttatcaccatcaaaatgagcaggggtcaggatatgcagccgacctgaagagcacacagaatgccattgacgagattactaacaaagtaaattctgttattgaaaagatgaatacacagttcacagcagtaggtaaagagttcaaccacctggaaaaaagaatagagaatttaaataaaaaagttgatgatggtttcctggacatttggacttacaatgccgaactgttggttctattggaaaatgaaagaactttggactaccacgattcaaatgtgaagaacttatatgaaaaggtaagaagccagctaaaaaacaatgccaaggaaattggaaacggctgctttgaattttaccacaaatgcgataacacgtgcatggaaagtgtcaaaaatgggacttatgactacccaaaatactcagaggaagcaaaattaaacagagaagaaatagatggggtaaagctggaatcaacaaggatttaccagattttggcgatctattcaactgtcgccagttcattggtactggtagtctccctgggggcaatcagtttctggatgtgctctaatgggtctctacagtgtagaatatgtatttaaaggcctattttctttagtttgaatttactgttattcggtgtgcatttctatgtttggtgagcggttttctgtgctcagagtgtgtttattttatgtaatttaatttctttgtgagctcctgtttagcaggtcgtcccttcagcaaggacacaaaaagattttaattttattaaaaaaaaaaaaaaaaaagaccgggaattcgatatcaagcttatcgacctgcagatcgttcaaacatttggcaataaagtttcttaagattgaatcctgttgccggtcttgcgatgattatcatataatttctgttgaattacgttaagcatgtaataattaacatgtaatgcatgacgttatttatgagatgggtttttatgattagagtcccgcaattatacatttaatacgcgatagaaaacaaaatatagcgcgcaaactaggataaattatcgcgcgcggtgtcatctatgttactagat

SEQ ID NO: 20 - protein, 573 aa, Influenza virus
MAKNVAIFGLLFSLLVLVPSQIFADTLCIGYHANNSTDTVDTVLEKNVTVTHSVNLLEDKHNGKLCKLRGVAPLHLGKCNIAGWILGNPECESLSTASSWSYIVETPSSDNGTCYPGDFIDYEELREQLSSVSSFERFEIFPKTSSWPNHDSNKGVTAACPHAGAKSFYKNLIWLVKKGNSYPKLSKSYINDKGKEVLVLWGIHHPSTSADQQSLYQNADAYVFVGSSRYSKKFKPEIAIRPKVRDQEGRMNYYWTLVEPGDKITFEATGNLVVPRYAFAMERNAGSGIIISDTPVHDCNTTCQTPKGAINTSLPFQNIHPITIGKCPKYVKSTKLRLATGLRNIPSIQSRGLFGAIAGFIEGGWTGMVDGWYGYHHQNEQGSGYAADLKSTQNAIDEITNKVNSVIEKMNTQFTAVGKEFNHLEKRIENLNKKVDDGFLDIWTYNAELLVLLENERTLDYHDSNVKNLYEKVRSQLKNNAKEIGNGCFEFYHKCDNTCMESVKNGTYDYPKYSEEAKLNREEIDGVKLESTRIYQILAIYSTVASSLVLVVSLGAISFWMCSNGSLQCRICI

SEQ ID NO: 21 - DNA, 40 bp, Artificial Sequence
  primer IF-S2+S4-H3 Per.c
tctcagatcttcgcccaaaaacttcctggaaatgacaaca

SEQ ID NO: 22 - DNA, 45 bp, Artificial Sequence
  primer IF-S1a4-H3 Per.r
actaaagaaaataggccttcaaatgcaaatgttgcacctaatgtt

SEQ ID NO: 23 - DNA, 1701 bp, Artificial Sequence
  nucleotide sequence of synthesized H3 gene
atgaagactatcattgctttgagctacattctatgtctggttttcgctcaaaaacttcctggaaatgacaacagcacggcaacgctgtgccttgggcaccatgcagtaccaaacggaacgatagtgaaaacaatcacgaatgaccaaattgaagttactaatgctactgagctggttcagagttcctcaacaggtgaaatatgcgacagtcctcatcagatccttgatggaaaaaactgcacactaatagatgctctattgggagaccctcagtgtgatggcttccaaaataagaaatgggacctttttgttgaacgcagcaaagcctacagcaactgttacccttatgatgtgccggattatgcctcccttaggtcactagttgcctcatccggcacactggagtttaacaatgaaagcttcaattggactggagtcactcaaaacggaacaagctctgcttgcataaggagatctaaaaacagtttctttagtagattgaattggttgacccacttaaacttcaaatacccagcattgaacgtgactatgccaaacaatgaacaatttgacaaattgtacatttggggggttcaccacccgggtacggacaaagaccaaatcttcctgtatgctcaagcatcaggaagaatcacagtctctaccaaaagaagccaacaaaccgtaagcccgaatatcggatctagacccagagtaaggaatatccctagcagaataagcatctattggacaatagtaaaaccgggagacatacttttgattaacagcacagggaatctaattgctcctaggggttacttcaaaatacgaagtgggaaaagctcaataatgagatcagatgcacccattggcaaatgcaattctgaatgcatcactccaaatggaagcattcccaatgacaaaccattccaaaatgtaaacaggatcacatacggggcctgtcccagatatgttaagcaaaacactctgaaattggcaacagggatgcgaaatgtaccagagaaacaaactagaggcatatttggcgcaatcgcgggtttcatagaaaatggttgggagggaatggtggatggttggtacggtttcaggcatcaaaattctgagggaagaggacaagcagcagatctcaaaagcactcaagcagcaatcgatcaaatcaatgggaagctgaatagattgatcgggaaaaccaacgagaaattccatcagattgaaaaagaattctcagaagtcgaagggagaattcaggaccttgagaaatatgttgaggacactaaaatagatctctggtcatacaacgcggagcttcttgttgccctggagaaccaacatacaattgatctaactgactcagaaatgaacaaactgtttgaaaaaacaaagaagcaactgagggaaaatgctgaggatatgggcaatggttgtttcaaaatataccacaaatgtgacaatgcctgcataggatcaatcagaaatggaacttatgaccacgatgtatacagagatgaagcattaaacaaccggtttcagatcaagggagttgagctgaagtcagggtacaaagattggatcctatggatttcctttgccatatcatgttttttgctttgtgttgctttgttggggttcatcatgtgggcctgccaaaaaggcaacattaggtgcaacatttgcatttga

SEQ ID NO: 24 - DNA, 3465 bp, Artificial Sequence
  Expression cassette number 1019
gtcaacatggtggagcacgacacacttgtctactccaaaaatatcaaagatacagtctcagaagaccaaagggcaattgagacttttcaacaaagggtaatatccggaaacctcctcggattccattgcccagctatctgtcactttattgtgaagatagtggaaaaggaaggtggctcctacaaatgccatcattgcgataaaggaaaggccatcgttgaagatgcctctgccgacagtggtcccaaagatggacccccacccacgaggagcatcgtggaaaaagaagacgttccaaccacgtcttcaaagcaagtggattgatgtgataacatggtggagcacgacacacttgtctactccaaaaatatcaaagatacagtctcagaagaccaaagggcaattgagacttttcaacaaagggtaatatccggaaacctcctcggattccattgcccagctatctgtcactttattgtgaagatagtggaaaaggaaggtggctcctacaaatgccatcattgcgataaaggaaaggccatcgttgaagatgcctctgccgacagtggtcccaaagatggacccccacccacgaggagcatcgtggaaaaagaagacgttccaaccacgtcttcaaagcaagtggattgatgtgatatctccactgacgtaagggatgacgcacaatcccactatccttcgcaagacccttcctctatataaggaagttcatttcatttggagaggtattaaaatcttaataggttttgataaaagcgaacgtggggaaacccgaaccaaaccttcttctaaactctctctcatctctcttaaagcaaacttctctcttgtctttcttgcgtgagcgatcttcaacgttgtcagatcgtgcttcggcaccagtacaacgttttctttcactgaagcgaaatcaaagatctctttgtggacacgtagtgcggcgccattaaataacgtgtacttgtcctattcttgtcggtgtggtcttgggaaaagaaagcttgctggaggctgctgttcagccccatacattacttgttacgattctgctgactttcggcgggtgcaatatctctacttctgcttgacgaggtattgttgcctgtacttctttcttcttcttcttgctgattggttctataagaaatctagtattttctttgaaacagagttttcccgtggttttcgaacttggagaaagattgttaagcttctgtatattctgcccaaatttgtcgggcccatggcgaaaaacgttgcgattttcggcttattgttttctcttcttgtgttggttccttctcagatcttcgcccaaaaacttcctggaaatgacaacagcacggcaacgctgtgccttgggcaccatgcagtaccaaacggaacgatagtgaaaacaatcacgaatgaccaaattgaagttactaatgctactgagctggttcagagttcctcaacaggtgaaatatgcgacagtcctcatcagatccttgatggaaaaaactgcacactaatagatgctctattgggagaccctcagtgtgatggcttccaaaataagaaatgggacctttttgttgaacgcagcaaagcctacagcaactgttacccttatgatgtgccggattatgcctcccttaggtcactagttgcctcatccggcacactggagtttaacaatgaaagcttcaattggactggagtcactcaaaacggaacaagctctgcttgcataaggagatctaaaaacagtttctttagtagattgaattggttgacccacttaaacttcaaatacccagcattgaacgtgactatgccaaacaatgaacaatttgacaaattgtacatttggggggttcaccacccgggtacggacaaagaccaaatcttcctgtatgctcaagcatcaggaagaatcacagtctctaccaaaagaagccaacaaaccgtaagcccgaatatcggatctagacccagagtaaggaatatccctagcagaataagcatctattggacaatagtaaaaccgggagacatacttttgattaacagcacagggaatctaattgctcctaggggttacttcaaaatacgaagtgggaaaagctcaataatgagatcagatgcacccattggcaaatgcaattctgaatgcatcactccaaatggaagcattcccaatgacaaaccattccaaaatgtaaacaggatcacatacggggcctgtcccagatatgttaagcaaaacactctgaaattggcaacagggatgcgaaatgtaccagagaaacaaactagaggcatatttggcgcaatcgcgggtttcatagaaaatggttgggagggaatggtggatggttggtacggtttcaggcatcaaaattctgagggaagaggacaagcagcagatctcaaaagcactcaagcagcaatcgatcaaatcaatgggaagctgaatagattgatcgggaaaaccaacgagaaattccatcagattgaaaaagaattctcagaagtcgaagggagaattcaggaccttgagaaatatgttgaggacactaaaatagatctctggtcatacaacgcggagcttcttgttgccctggagaaccaacatacaattgatctaactgactcagaaatgaacaaactgtttgaaaaaacaaagaagcaactgagggaaaatgctgaggatatgggcaatggttgtttcaaaatataccacaaatgtgacaatgcctgcataggatcaatcagaaatggaacttatgaccacgatgtatacagagatgaagcattaaacaaccggtttcagatcaagggagttgagctgaagtcagggtacaaagattggatcctatggatttcctttgccatatcatgttttttgctttgtgttgctttgttggggttcatcatgtgggcctgccaaaaaggcaacattaggtgcaacatttgcatttgaaggcctattttctttagtttgaatttactgttattcggtgtgcatttctatgtttggtgagcggttttctgtgctcagagtgtgtttattttatgtaatttaatttctttgtgagctcctgtttagcaggtcgtcccttcagcaaggacacaaaaagattttaattttattaaaaaaaaaaaaaaaaaagaccgggaattcgatatcaagcttatcgacctgcagatcgttcaaacatttggcaataaagtttcttaagattgaatcctgttgccggtcttgcgatgattatcatataatttctgttgaattacgttaagcatgtaataattaacatgtaatgcatgacgttatttatgagatgggtttttatgattagagtcccgcaattatacatttaatacgcgatagaaaacaaaatatagcgcgcaaactaggataaattatcgcgcgcggtgtcatctatgttactagat

SEQ ID NO: 25 - protein, 574 aa, Influenza virus
MAKNVAIFGLLFSLLVLVPSQIFAQKLPGNDNSTATLCLGHHAVPNGTIVKTITNDQIEVTNATELVQSSSTGEICDSPHQILDGKNCTLIDALLGDPQCDGFQNKKWDLFVERSKAYSNCYPYDVPDYASLRSLVASSGTLEFNNESFNWTGVTQNGTSSACIRRSKNSFFSRLNWLTHLNFKYPALNVTMPNNEQFDKLYIWGVHHPGTDKDQIFLYAQASGRITVSTKRSQQTVSPNIGSRPRVRNIPSRISIYWTIVKPGDILLINSTGNLIAPRGYFKIRSGKSSIMRSDAPIGKCNSECITPNGSIPNDKPFQNVNRITYGACPRYVKQNTLKLATGMRNVPEKQTRGIFGAIAGFIENGWEGMVDGWYGFRHQNSEGRGQAADLKSTQAAIDQINGKLNRLIGKTNEKFHQIEKEFSEVEGRIQDLEKYVEDTKIDLWSYNAELLVALENQHTIDLTDSEMNKLFEKTKKQLRENAEDMGNGCFKIYHKCDNACIGSIRNGTYDHDVYRDEALNNRFQIKGVELKSGYKDWILWISFAISCFLLCVALLGFIMWACQKGNIRCNICI

SEQ ID NO: 26 - DNA, 40 bp, Artificial Sequence
  primer IF-S2+S4-B Bris.c
tctcagatcttcgccgatcgaatctgcactggaataacat

SEQ ID NO: 27 - DNA, 43 bp, Artificial Sequence
  primer IF-S1a4-B Bris.r
actaaagaaaataggcctttatagacagatggagcaagaaaca

SEQ ID NO: 28 - DNA, 1758 bp, Artificial Sequence
  nucleotide sequence of synthesized HA B Brisbane gene
atgaaggcaataattgtactactcatggtagtaacatccaatgcagatcgaatctgcactggaataacatcgtcaaactcaccacatgtcgtcaaaactgctactcaaggggaggtcaatgtgactggtgtaataccactgacaacaacacccaccaaatctcattttgcaaatctcaaaggaacagaaaccagggggaaactatgcccaaaatgcctcaactgcacagatctggacgtagccttgggcagaccaaaatgcacggggaaaataccctcggcaagagtttcaatactccatgaagtcagacctgttacatctgggtgctttcctataatgcacgacagaacaaaaattagacagctgcctaaccttctccgaggatacgaacatatcaggttatcaacccataacgttatcaatgcagaaaatgcaccaggaggaccctacaaaattggaacctcagggtcttgccctaacattaccaatggaaacggatttttcgcaacaatggcttgggccgtcccaaaaaacgacaaaaacaaaacagcaacaaatccattaacaatagaagtaccatacatttgtacagaaggagaagaccaaattaccgtttgggggttccactctgacaacgagacccaaatggcaaagctctatggggactcaaagccccagaagttcacctcatctgccaacggagtgaccacacattacgtttcacagattggtggcttcccaaatcaaacagaagacggaggactaccacaaagtggtagaattgttgttgattacatggtgcaaaaatctgggaaaacaggaacaattacctatcaaaggggtattttattgcctcaaaaggtgtggtgcgcaagtggcaggagcaaggtaataaaaggatccttgcctttaattggagaagcagattgcctccacgaaaaatacggtggattaaacaaaagcaagccttactacacaggggaacatgcaaaggccataggaaattgcccaatatgggtgaaaacacccttgaagctggccaatggaaccaaatatagacctcctgcaaaactattaaaggaaaggggtttcttcggagctattgctggtttcttagaaggaggatgggaaggaatgattgcaggttggcacggatacacatcccatggggcacatggagtagcggtggcagcagaccttaagagcactcaagaggccataaacaagataacaaaaaatctcaactctttgagtgagctggaagtaaagaatcttcaaagactaagcggtgccatggatgaactccacaacgaaatactagaactagatgagaaagtggatgatctcagagctgatacaataagctcacaaatagaactcgcagtcctgctttccaatgaaggaataataaacagtgaagatgaacatctcttggcgcttgaaagaaagctgaagaaaatgctgggcccctctgctgtagagatagggaatggatgctttgaaaccaaacacaagtgcaaccagacctgtctcgacagaatagctgctggtacctttgatgcaggagaattttctctccccacctttgattcactgaatattactgctgcatctttaaatgacgatggattggataatcatactatactgctttactactcaactgctgcctccagtttggctgtaacactgatgatagctatctttgttgtttatatggtctccagagacaatgtttcttgctccatctgtctataa

SEQ ID NO: 29 - DNA, 3525 bp, Artificial Sequence
  Expression cassette number 1029
gtcaacatggtggagcacgacacacttgtctactccaaaaatatcaaagatacagtctcagaagaccaaagggcaattgagacttttcaacaaagggtaatatccggaaacctcctcggattccattgcccagctatctgtcactttattgtgaagatagtggaaaaggaaggtggctcctacaaatgccatcattgcgataaaggaaaggccatcgttgaagatgcctctgccgacagtggtcccaaagatggacccccacccacgaggagcatcgtggaaaaagaagacgttccaaccacgtcttcaaagcaagtggattgatgtgataacatggtggagcacgacacacttgtctactccaaaaatatcaaagatacagtctcagaagaccaaagggcaattgagacttttcaacaaagggtaatatccggaaacctcctcggattccattgcccagctatctgtcactttattgtgaagatagtggaaaaggaaggtggctcctacaaatgccatcattgcgataaaggaaaggccatcgttgaagatgcctctgccgacagtggtcccaaagatggacccccacccacgaggagcatcgtggaaaaagaagacgttccaaccacgtcttcaaagcaagtggattgatgtgatatctccactgacgtaagggatgacgcacaatcccactatccttcgcaagacccttcctctatataaggaagttcatttcatttggagaggtattaaaatcttaataggttttgataaaagcgaacgtggggaaacccgaaccaaaccttcttctaaactctctctcatctctcttaaagcaaacttctctcttgtctttcttgcgtgagcgatcttcaacgttgtcagatcgtgcttcggcaccagtacaacgttttctttcactgaagcgaaatcaaagatctctttgtggacacgtagtgcggcgccattaaataacgtgtacttgtcctattcttgtcggtgtggtcttgggaaaagaaagcttgctggaggctgctgttcagccccatacattacttgttacgattctgctgactttcggcgggtgcaatatctctacttctgcttgacgaggtattgttgcctgtacttctttcttcttcttcttgctgattggttctataagaaatctagtattttctttgaaacagagttttcccgtggttttcgaacttggagaaagattgttaagcttctgtatattctgcccaaatttgtcgggcccatggcgaaaaacgttgcgattttcggcttattgttttctcttcttgtgttggttccttctcagatcttcgccgatcgaatctgcactggaataacatcgtcaaactcaccacatgtcgtcaaaactgctactcaaggggaggtcaatgtgactggtgtaataccactgacaacaacacccaccaaatctcattttgcaaatctcaaaggaacagaaaccagggggaaactatgcccaaaatgcctcaactgcacagatctggacgtagccttgggcagaccaaaatgcacggggaaaataccctcggcaagagtttcaatactccatgaagtcagacctgttacatctgggtgctttcctataatgcacgacagaacaaaaattagacagctgcctaaccttctccgaggatacgaacatatcaggttatcaacccataacgttatcaatgcagaaaatgcaccaggaggaccctacaaaattggaacctcagggtcttgccctaacattaccaatggaaacggatttttcgcaacaatggcttgggccgtcccaaaaaacgacaaaaacaaaacagcaacaaatccattaacaatagaagtaccatacatttgtacagaaggagaagaccaaattaccgtttgggggttccactctgacaacgagacccaaatggcaaagctctatggggactcaaagccccagaagttcacctcatctgccaacggagtgaccacacattacgtttcacagattggtggcttcccaaatcaaacagaagacggaggactaccacaaagtggtagaattgttgttgattacatggtgcaaaaatctgggaaaacaggaacaattacctatcaaaggggtattttattgcctcaaaaggtgtggtgcgcaagtggcaggagcaaggtaataaaaggatccttgcctttaattggagaagcagattgcctccacgaaaaatacggtggattaaacaaaagcaagccttactacacaggggaacatgcaaaggccataggaaattgcccaatatgggtgaaaacacccttgaagctggccaatggaaccaaatatagacctcctgcaaaactattaaaggaaaggggtttcttcggagctattgctggtttcttagaaggaggatgggaaggaatgattgcaggttggcacggatacacatcccatggggcacatggagtagcggtggcagcagaccttaagagcactcaagaggccataaacaagataacaaaaaatctcaactctttgagtgagctggaagtaaagaatcttcaaagactaagcggtgccatggatgaactccacaacgaaatactagaactagatgagaaagtggatgatctcagagctgatacaataagctcacaaatagaactcgcagtcctgctttccaatgaaggaataataaacagtgaagatgaacatctcttggcgcttgaaagaaagctgaagaaaatgctgggcccctctgctgtagagatagggaatggatgctttgaaaccaaacacaagtgcaaccagacctgtctcgacagaatagctgctggtacctttgatgcaggagaattttctctccccacctttgattcactgaatattactgctgcatctttaaatgacgatggattggataatcatactatactgctttactactcaactgctgcctccagtttggctgtaacactgatgatagctatctttgttgtttatatggtctccagagacaatgtttcttgctccatctgtctataaaggcctattttctttagtttgaatttactgttattcggtgtgcatttctatgtttggtgagcggttttctgtgctcagagtgtgtttattttatgtaatttaatttctttgtgagctcctgtttagcaggtcgtcccttcagcaaggacacaaaaagattttaattttattaaaaaaaaaaaaaaaaaagaccgggaattcgatatcaagcttatcgacctgcagatcgttcaaacatttggcaataaagtttcttaagattgaatcctgttgccggtcttgcgatgattatcatataatttctgttgaattacgttaagcatgtaataattaacatgtaatgcatgacgttatttatgagatgggtttttatgattagagtcccgcaattatacatttaatacgcgatagaaaacaaaatatagcgcgcaaactaggataaattatcgcgcgcggtgtcatctatgttactagat

SEQ ID NO: 30 - protein, 594 aa, Influenza virus
MAKNVAIFGLLFSLLVLVPSQIFADRICTGITSSNSPHVVKTATQGEVNVTGVIPLTTTPTKSHFANLKGTETRGKLCPKCLNCTDLDVALGRPKCTGKIPSARVSILHEVRPVTSGCFPIMHDRTKIRQLPNLLRGYEHIRLSTHNVINAENAPGGPYKIGTSGSCPNITNGNGFFATMAWAVPKNDKNKTATNPLTIEVPYICTEGEDQITVWGFHSDNETQMAKLYGDSKPQKFTSSANGVTTHYVSQIGGFPNQTEDGGLPQSGRIVVDYMVQKSGKTGTITYQRGILLPQKVWCASGRSKVIKGSLPLIGEADCLHEKYGGLNKSKPYYTGEHAKAIGNCPIWVKTPLKLANGTKYRPPAKLLKERGFFGAIAGFLEGGWEGMIAGWHGYTSHGAHGVAVAADLKSTQEAINKITKNLNSLSELEVKNLQRLSGAMDELHNEILELDEKVDDLRADTISSQIELAVLLSNEGIINSEDEHLLALERKLKKMLGPSAVEIGNGCFETKHKCNQTCLDRIAAGTFDAGEFSLPTFDSLNITAASLNDDGLDNHTILLYYSTAASSLAVTLMIAIFVVYMVSRDNVSCSICL

SEQ ID NO: 31 - DNA, 6861 bp, Artificial Sequence
  Construct 1194
tggcaggatatattgtggtgtaaacaaattgacgcttagacaacttaataacacattgcggacgtttttaatgtactgaattaacgccgaatcccgggctggtatatttatatgttgtcaaataactcaaaaaccataaaagtttaagttagcaagtgtgtacatttttacttgaacaaaaatattcacctactactgttataaatcattattaaacattagagtaaagaaatatggatgataagaacaagagtagtgatattttgacaacaattttgttgcaacatttgagaaaattttgttgttctctcttttcattggtcaaaaacaatagagagagaaaaaggaagagggagaataaaaacataatgtgagtatgagagagaaagttgtacaaaagttgtaccaaaatagttgtacaaatatcattgaggaatttgacaaaagctacacaaataagggttaattgctgtaaataaataaggatgacgcattagagagatgtaccattagagaatttttggcaagtcattaaaaagaaagaataaattatttttaaaattaaaagttgagtcatttgattaaacatgtgattatttaatgaattgatgaaagagttggattaaagttgtattagtaattagaatttggtgtcaaatttaatttgacatttgatcttttcctatatattgccccatagagtcagttaactcatttttatatttcatagatcaaataagagaaataacggtatattaatccctccaaaaaaaaaaaacggtatatttactaaaaaatctaagccacgtaggaggataacaggatccccgtaggaggataacatccaatccaaccaatcacaacaatcctgatgagataacccactttaagcccacgcatctgtggcacatctacattatctaaatcacacattcttccacacatctgagccacacaaaaaccaatccacatctttatcacccattctataaaaaatcacactttgtgagtctacactttgattcccttcaaacacatacaaagagaagagactaattaattaattaatcatcttgagagaaaatggaacgagctatacaaggaaacgacgctagggaacaagctaacagtgaacgttgggatggaggatcaggaggtaccacttctcccttcaaacttcctgacgaaagtccgagttggactgagtggcggctacataacgatgagacgaattcgaatcaagataatccccttggtttcaaggaaagctggggtttcgggaaagttgtatttaagagatatctcagatacgacaggacggaagcttcactgcacagagtccttggatcttggacgggagattcggttaactatgcagcatctcgatttttcggtttcgaccagatcggatgtacctatagtattcggtttcgaggagttagtatcaccgtttctggagggtcgcgaactcttcagcatctctgtgagatggcaattcggtctaagcaagaactgctacagcttgccccaatcgaagtggaaagtaatgtatcaagaggatgccctgaaggtactcaaaccttcgaaaaagaaagcgagtaagttaaaatgcttcttcgtctcctatttataatatggtttgttattgttaattttgttcttgtagaagagcttaattaatcgttgttgttatgaaatactatttgtatgagatgaactggtgtaatgtaattcatttacataagtggagtcagaatcagaatgtttcctccataactaactagacatgaagacctgccgcgtacaattgtcttatatttgaacaactaaaattgaacatcttttgccacaactttataagtggttaatatagctcaaatatatggtcaagttcaatagattaataatggaaatatcagttatcgaaattcattaacaatcaacttaacgttattaactactaattttatatcatcccctttgataaatgatagtacaccaattaggaaggagcatgctcgcctaggagattgtcgtttcccgccttcagtttgcaagctgctctagccgtgtagccaatacgcaaaccgcctctccccgcgcgttgggaattactagcgcgtgtcgacacgcgtggcgcgccctagcagaaggcatgttgttgtgactccgaggggttgcctcaaactctatcttataaccggcgtggaggcatggaggcaagggcattttggtaatttaagtagttagtggaaaatgacgtcatttacttaaagacgaagtcttgcgacaaggggggcccacgccgaattttaatattaccggcgtggccccaccttatcgcgagtgctttagcacgagcggtccagatttaaagtagaaaagttcccgcccactagggttaaaggtgttcacactataaaagcatatacgatgtgatggtatttgataaagcgtatattgtatcaggtatttccgtcggatacgaattattcgtacaagcttcttaagccggtcaacatggtggagcacgacacacttgtctactccaaaaatatcaaagatacagtctcagaagaccaaagggcaattgagacttttcaacaaagggtaatatccggaaacctcctcggattccattgcccagctatctgtcactttattgtgaagatagtggaaaaggaaggtggctcctacaaatgccatcattgcgataaaggaaaggccatcgttgaagatgcctctgccgacagtggtcccaaagatggacccccacccacgaggagcatcgtggaaaaagaagacgttccaaccacgtcttcaaagcaagtggattgatgtgataacatggtggagcacgacacacttgtctactccaaaaatatcaaagatacagtctcagaagaccaaagggcaattgagacttttcaacaaagggtaatatccggaaacctcctcggattccattgcccagctatctgtcactttattgtgaagatagtggaaaaggaaggtggctcctacaaatgccatcattgcgataaaggaaaggccatcgttgaagatgcctctgccgacagtggtcccaaagatggacccccacccacgaggagcatcgtggaaaaagaagacgttccaaccacgtcttcaaagcaagtggattgatgtgatatctccactgacgtaagggatgacgcacaatcccactatccttcgcaagacccttcctctatataaggaagttcatttcatttggagaggtattaaaatcttaataggttttgataaaagcgaacgtggggaaacccgaaccaaaccttcttctaaactctctctcatctctcttaaagcaaacttctctcttgtctttcttgcgtgagcgatcttcaacgttgtcagatcgtgcttcggcaccagtacaacgttttctttcactgaagcgaaatcaaagatctctttgtggacacgtagtgcggcgccattaaataacgtgtacttgtcctattcttgtcggtgtggtcttgggaaaagaaagcttgctggaggctgctgttcagccccatacattacttgttacgattctgctgactttcggcgggtgcaatatctctacttctgcttgacgaggtattgttgcctgtacttctttcttcttcttcttgctgattggttctataagaaatctagtattttctttgaaacagagttttcccgtggttttcgaacttggagaaagattgttaagcttctgtatattctgcccaaatttgtcgggcccatggcgaaaaacgttgcgattttcggcttattgttttctcttcttgtgttggttccttctcagatcttcgccgcggctcctcagccaaaacgacacccccatctgtctatccactggcccctggatctgctgcccaaactaactccatggtgaccctgggatgcctggtcaagggctatttccctgagccagtgacagtgacctggaactctggatccctgtccagcggtgtgcacaccttcccagctgtcctgcagtctgacctctacactctgagcagctcagtgactgtcccctccagcacctggcccagcgagaccgtcacctgcaacgttgcccacccggccagcagcaccaaggtggacaagaaaattgtgcccagggattgtggttgtaagccttgcatatgtacagtcccagaagtatcatctgtcttcatcttccccccaaagcccaaggatgtgctcaccattactctgactcctaaggtcacgtgtgttgtggtagacatcagcaaggatgatcccgaggtccagttcagctggtttgtagatgatgtggaggtgcacacagctcagacgcaaccccgggaggagcagttcaacagcactttccgctcagtcagtgaacttcccatcatgcaccaggactggctcaatggcaaggaaggcctattttctttagtttgaatttactgttattcggtgtgcatttctatgtttggtgagcggttttctgtgctcagagtgtgtttattttatgtaatttaatttctttgtgagctcctgtttagcaggtcgtcccttcagcaaggacacaaaaagattttaattttattaaaaaaaaaaaaaaaaaagaccgggaattcgatatcaagcttatcgacctgcagatcgttcaaacatttggcaataaagtttcttaagattgaatcctgttgccggtcttgcgatgattatcatataatttctgttgaattacgttaagcatgtaataattaacatgtaatgcatgacgttatttatgagatgggtttttatgattagagtcccgcaattatacatttaatacgcgatagaaaacaaaatatagcgcgcaaactaggataaattatcgcgcgcggtgtcatctatgttactagatctctagagtctcaagcttggcgcggggtaccgagctcgaattccgagtgtacttcaagtcagttggaaatcaataaaatgattattttatgaatatatttcattgtgcaagtagatagaaattacatatgttacataacacacgaaataaacaaaaaaacacaatccaaaacaaacaccccaaacaaaataacactatatatatcctcgtatgaggagaggcacgttcagtgactcgacgattcccgagcaaaaaaagtctccccgtcacacatatagtgggtgacgcaattatcttcaaagtaatccttctgttgacttgtcattgataacatccagtcttcgtcaggattgcaaagaattatagaagggatcccaccttttattttcttcttttttccatatttagggttgacagtgaaatcagactggcaacctattaattgcttccacaatgggacgaacttgaaggggatgtcgtcgatgatattataggtggcgtgttcatcgtagttggtgaagtcgatggtcccgttccagtagttgtgtcgcccgagacttctagcccaggtggtctttccggtacgagttggtccgcagatgtagaggctggggtgtctgaccccagtccttccctcatcctggttagatcggccatccactcaaggtcagattgtgcttgatcgtaggagacaggatgtatgaaagtgtaggcatcgatgcttacatgatataggtgcgtctctctccagttgtgcagatcttcgtggcagcggagatctgattctgtgaagggcgacacgtactgctcaggttgtggaggaaataatttgttggctgaatattccagccattgaagctttgttgcccattcatgagggaattcttctttgatcatgtcaagatactcctccttagacgttgcagtctggataatagttcgccatcgtgcgtcagatttgcgaggagagaccttatgatctcggaaatctcctctggttttaatatctccgtcctttgatatgtaatcaaggacttgtttagagtttctagctggctggatattagggtgatttccttcaaaatcgaaaaaagaaggatccctaatacaaggttttttatcaagctggataagagcatgatagtgggtagtgccatcttgatgaagctcagaagcaacaccaaggaagaaaataagaaaaggtgtgagtttctcccagagaaactggaataaatcatctctttgagatgagcacttggggtaggtaaggaaaacatatttagattggagtctgaagttcttgctagcagaaggcatgttgttgtgactccgaggggttgcctcaaactctatcttataaccggcgtggaggcatggaggcaagggcattttggtaatttaagtagttagtggaaaatgacgtcatttacttaaagacgaagtcttgcgacaaggggggcccacgccgaattttaatattaccggcgtggccccaccttatcgcgagtgctttagcacgagcggtccagatttaaagtagaaaagttcccgcccactagggttaaaggtgttcacactataaaagcatatacgatgtgatggtatttgatggagcgtatattgtatcaggtatttccgtcggatacgaattattcgtacggccggccactagtggcactggccgtcgttttacaacgtcgtgactgggaaaaccctggcgttacccaacttaatcgccttgcagcacatccccctttcgccagctggcgtaatagcgaagaggcccgcaccgatcgcccttcccaacagttgcgcagcctgaatggcgaatgctagagcagcttgagcttggatcagattgtcgtttcccgccttcagtttaaactatcagtgtttgacaggatatattggcgggtaaacctaagagaaaagagcgttta

SEQ ID NO: 32 - DNA, 5555 bp, Artificial Sequence
  Expression cassette number 1008
ctagcagaaggcatgttgttgtgactccgaggggttgcctcaaactctatcttataaccggcgtggaggcatggaggcaagggcattttggtaatttaagtagttagtggaaaatgacgtcatttacttaaagacgaagtcttgcgacaaggggggcccacgccgaattttaatattaccggcgtggccccaccttatcgcgagtgctttagcacgagcggtccagatttaaagtagaaaagttcccgcccactagggttaaaggtgttcacactataaaagcatatacgatgtgatggtatttgataaagcgtatattgtatcaggtatttccgtcggatacgaattattcgtacaagcttcttaagccggtcaacatggtggagcacgacacacttgtctactccaaaaatatcaaagatacagtctcagaagaccaaagggcaattgagacttttcaacaaagggtaatatccggaaacctcctcggattccattgcccagctatctgtcactttattgtgaagatagtggaaaaggaaggtggctcctacaaatgccatcattgcgataaaggaaaggccatcgttgaagatgcctctgccgacagtggtcccaaagatggacccccacccacgaggagcatcgtggaaaaagaagacgttccaaccacgtcttcaaagcaagtggattgatgtgataacatggtggagcacgacacacttgtctactccaaaaatatcaaagatacagtctcagaagaccaaagggcaattgagacttttcaacaaagggtaatatccggaaacctcctcggattccattgcccagctatctgtcactttattgtgaagatagtggaaaaggaaggtggctcctacaaatgccatcattgcgataaaggaaaggccatcgttgaagatgcctctgccgacagtggtcccaaagatggacccccacccacgaggagcatcgtggaaaaagaagacgttccaaccacgtcttcaaagcaagtggattgatgtgatatctccactgacgtaagggatgacgcacaatcccactatccttcgcaagacccttcctctatataaggaagttcatttcatttggagaggtattaaaatcttaataggttttgataaaagcgaacgtggggaaacccgaaccaaaccttcttctaaactctctctcatctctcttaaagcaaacttctctcttgtctttcttgcgtgagcgatcttcaacgttgtcagatcgtgcttcggcaccagtacaacgttttctttcactgaagcgaaatcaaagatctctttgtggacacgtagtgcggcgccattaaataacgtgtacttgtcctattcttgtcggtgtggtcttgggaaaagaaagcttgctggaggctgctgttcagccccatacattacttgttacgattctgctgactttcggcgggtgcaatatctctacttctgcttgacgaggtattgttgcctgtacttctttcttcttcttcttgctgattggttctataagaaatctagtattttctttgaaacagagttttcccgtggttttcgaacttggagaaagattgttaagcttctgtatattctgcccaaatttgtcgggcccatggcgaaaaacgttgcgattttcggcttattgttttctcttcttgtgttggttccttctcagatcttcgccgatcgaatctgcactggaataacatcgtcaaactcaccacatgtcgtcaaaactgctactcaaggggaggtcaatgtgactggtgtaataccactgacaacaacacccaccaaatctcattttgcaaatctcaaaggaacagaaaccagggggaaactatgcccaaaatgcctcaactgcacagatctggacgtagccttgggcagaccaaaatgcacggggaaaataccctcggcaagagtttcaatactccatgaagtcagacctgttacatctgggtgctttcctataatgcacgacagaacaaaaattagacagctgcctaaccttctccgaggatacgaacatatcaggttatcaacccataacgttatcaatgcagaaaatgcaccaggaggaccctacaaaattggaacctcagggtcttgccctaacattaccaatggaaacggatttttcgcaacaatggcttgggccgtcccaaaaaacgacaaaaacaaaacagcaacaaatccattaacaatagaagtaccatacatttgtacagaaggagaagaccaaattaccgtttgggggttccactctgacaacgagacccaaatggcaaagctctatggggactcaaagccccagaagttcacctcatctgccaacggagtgaccacacattacgtttcacagattggtggcttcccaaatcaaacagaagacggaggactaccacaaagtggtagaattgttgttgattacatggtgcaaaaatctgggaaaacaggaacaattacctatcaaaggggtattttattgcctcaaaaggtgtggtgcgcaagtggcaggagcaaggtaataaaaggatccttgcctttaattggagaagcagattgcctccacgaaaaatacggtggattaaacaaaagcaagccttactacacaggggaacatgcaaaggccataggaaattgcccaatatgggtgaaaacacccttgaagctggccaatggaaccaaatatagacctcctgcaaaactattaaaggaaaggggtttcttcggagctattgctggtttcttagaaggaggatgggaaggaatgattgcaggttggcacggatacacatcccatggggcacatggagtagcggtggcagcagaccttaagagcactcaagaggccataaacaagataacaaaaaatctcaactctttgagtgagctggaagtaaagaatcttcaaagactaagcggtgccatggatgaactccacaacgaaatactagaactagatgagaaagtggatgatctcagagctgatacaataagctcacaaatagaactcgcagtcctgctttccaatgaaggaataataaacagtgaagatgaacatctcttggcgcttgaaagaaagctgaagaaaatgctgggcccctctgctgtagagatagggaatggatgctttgaaaccaaacacaagtgcaaccagacctgtctcgacagaatagctgctggtacctttgatgcaggagaattttctctccccacctttgattcactgaatattactgctgcatctttaaatgacgatggattggataatcatactatactgctttactactcaactgctgcctccagtttggctgtaacactgatgatagctatctttgttgtttatatggtctccagagacaatgtttcttgctccatctgtctataaaggcctattttctttagtttgaatttactgttattcggtgtgcatttctatgtttggtgagcggttttctgtgctcagagtgtgtttattttatgtaatttaatttctttgtgagctcctgtttagcaggtcgtcccttcagcaaggacacaaaaagattttaattttattaaaaaaaaaaaaaaaaaagaccgggaattcgatatcaagcttatcgacctgcagatcgttcaaacatttggcaataaagtttcttaagattgaatcctgttgccggtcttgcgatgattatcatataatttctgttgaattacgttaagcatgtaataattaacatgtaatgcatgacgttatttatgagatgggtttttatgattagagtcccgcaattatacatttaatacgcgatagaaaacaaaatatagcgcgcaaactaggataaattatcgcgcgcggtgtcatctatgttactagatctctagagtctcaagcttggcgcggggtaccgagctcgaattccgagtgtacttcaagtcagttggaaatcaataaaatgattattttatgaatatatttcattgtgcaagtagatagaaattacatatgttacataacacacgaaataaacaaaaaaacacaatccaaaacaaacaccccaaacaaaataacactatatatatcctcgtatgaggagaggcacgttcagtgactcgacgattcccgagcaaaaaaagtctccccgtcacacatatagtgggtgacgcaattatcttcaaagtaatccttctgttgacttgtcattgataacatccagtcttcgtcaggattgcaaagaattatagaagggatcccaccttttattttcttcttttttccatatttagggttgacagtgaaatcagactggcaacctattaattgcttccacaatgggacgaacttgaaggggatgtcgtcgatgatattataggtggcgtgttcatcgtagttggtgaagtcgatggtcccgttccagtagttgtgtcgcccgagacttctagcccaggtggtctttccggtacgagttggtccgcagatgtagaggctggggtgtctgaccccagtccttccctcatcctggttagatcggccatccactcaaggtcagattgtgcttgatcgtaggagacaggatgtatgaaagtgtaggcatcgatgcttacatgatataggtgcgtctctctccagttgtgcagatcttcgtggcagcggagatctgattctgtgaagggcgacacgtactgctcaggttgtggaggaaataatttgttggctgaatattccagccattgaagctttgttgcccattcatgagggaattcttctttgatcatgtcaagatactcctccttagacgttgcagtctggataatagttcgccatcgtgcgtcagatttgcgaggagagaccttatgatctcggaaatctcctctggttttaatatctccgtcctttgatatgtaatcaaggacttgtttagagtttctagctggctggatattagggtgatttccttcaaaatcgaaaaaagaaggatccctaatacaaggttttttatcaagctggataagagcatgatagtgggtagtgccatcttgatgaagctcagaagcaacaccaaggaagaaaataagaaaaggtgtgagtttctcccagagaaactggaataaatcatctctttgagatgagcacttggggtaggtaaggaaaacatatttagattggagtctgaagttcttgctagcagaaggcatgttgttgtgactccgaggggttgcctcaaactctatcttataaccggcgtggaggcatggaggcaagggcattttggtaatttaagtagttagtggaaaatgacgtcatttacttaaagacgaagtcttgcgacaaggggggcccacgccgaattttaatattaccggcgtggccccaccttatcgcgagtgctttagcacgagcggtccagatttaaagtagaaaagttcccgcccactagggttaaaggtgttcacactataaaagcatatacgatgtgatggtatttgatggagcgtatattgtatcaggtatttccgtcggatacgaattattcgtac

SEQ ID NO: 33 - DNA, 50 bp, Artificial Sequence
  primer dTmH5I-B Bris.r
ttgacagtatttggtaattatccaatccatcgtcatttaaagatgcagca

SEQ ID NO: 34 - DNA, 50 bp, Artificial Sequence
  primer B Bris-dTmH5I.c
catctttaaatgacgatggattggataattaccaaatactgtcaatttat

SEQ ID NO: 35 - DNA, 50 bp, Artificial Sequence; identical to SEQ ID NO: 3
  primer IF-S1aS4-dTmH5I.r

SEQ ID NO: 36 - DNA, 5555 bp, Artificial Sequence
  Expression cassette number 1009
ctagcagaaggcatgttgttgtgactccgaggggttgcctcaaactctatcttataaccggcgtggaggcatggaggcaagggcattttggtaatttaagtagttagtggaaaatgacgtcatttacttaaagacgaagtcttgcgacaaggggggcccacgccgaattttaatattaccggcgtggccccaccttatcgcgagtgctttagcacgagcggtccagatttaaagtagaaaagttcccgcccactagggttaaaggtgttcacactataaaagcatatacgatgtgatggtatttgataaagcgtatattgtatcaggtatttccgtcggatacgaattattcgtacaagcttcttaagccggtcaacatggtggagcacgacacacttgtctactccaaaaatatcaaagatacagtctcagaagaccaaagggcaattgagacttttcaacaaagggtaatatccggaaacctcctcggattccattgcccagctatctgtcactttattgtgaagatagtggaaaaggaaggtggctcctacaaatgccatcattgcgataaaggaaaggccatcgttgaagatgcctctgccgacagtggtcccaaagatggacccccacccacgaggagcatcgtggaaaaagaagacgttccaaccacgtcttcaaagcaagtggattgatgtgataacatggtggagcacgacacacttgtctactccaaaaatatcaaagatacagtctcagaagaccaaagggcaattgagacttttcaacaaagggtaatatccggaaacctcctcggattccattgcccagctatctgtcactttattgtgaagatagtggaaaaggaaggtggctcctacaaatgccatcattgcgataaaggaaaggccatcgttgaagatgcctctgccgacagtggtcccaaagatggacccccacccacgaggagcatcgtggaaaaagaagacgttccaaccacgtcttcaaagcaagtggattgatgtgatatctccactgacgtaagggatgacgcacaatcccactatccttcgcaagacccttcctctatataaggaagttcatttcatttggagaggtattaaaatcttaataggttttgataaaagcgaacgtggggaaacccgaaccaaaccttcttctaaactctctctcatctctcttaaagcaaacttctctcttgtctttcttgcgtgagcgatcttcaacgttgtcagatcgtgcttcggcaccagtacaacgttttctttcactgaagcgaaatcaaagatctctttgtggacacgtagtgcggcgccattaaataacgtgtacttgtcctattcttgtcggtgtggtcttgggaaaagaaagcttgctggaggctgctgttcagccccatacattacttgttacgattctgctgactttcggcgggtgcaatatctctacttctgcttgacgaggtattgttgcctgtacttctttcttcttcttcttgctgattggttctataagaaatctagtattttctttgaaacagagttttcccgtggttttcgaacttggagaaagattgttaagcttctgtatattctgcccaaatttgtcgggcccatggcgaaaaacgttgcgattttcggcttattgttttctcttcttgtgttggttccttctcagatcttcgccgatcgaatctgcactggaataacatcgtcaaactcaccacatgtcgtcaaaactgctactcaaggggaggtcaatgtgactggtgtaataccactgacaacaacacccaccaaatctcattttgcaaatctcaaaggaacagaaaccagggggaaactatgcccaaaatgcctcaactgcacagatctggacgtagccttgggcagaccaaaatgcacggggaaaataccctcggcaagagtttcaatactccatgaagtcagacctgttacatctgggtgctttcctataatgcacgacagaacaaaaattagacagctgcctaaccttctccgaggatacgaacatatcaggttatcaacccataacgttatcaatgcagaaaatgcaccaggaggaccctacaaaattggaacctcagggtcttgccctaacattaccaatggaaacggatttttcgcaacaatggcttgggccgtcccaaaaaacgacaaaaacaaaacagcaacaaatccattaacaatagaagtaccatacatttgtacagaaggagaagaccaaattaccgtttgggggttccactctgacaacgagacccaaatggcaaagctctatggggactcaaagccccagaagttcacctcatctgccaacggagtgaccacacattacgtttcacagattggtggcttcccaaatcaaacagaagacggaggactaccacaaagtggtagaattgttgttgattacatggtgcaaaaatctgggaaaacaggaacaattacctatcaaaggggtattttattgcctcaaaaggtgtggtgcgcaagtggcaggagcaaggtaataaaaggatccttgcctttaattggagaagcagattgcctccacgaaaaatacggtggattaaacaaaagcaagccttactacacaggggaacatgcaaaggccataggaaattgcccaatatgggtgaaaacacccttgaagctggccaatggaaccaaatatagacctcctgcaaaactattaaaggaaaggggtttcttcggagctattgctggtttcttagaaggaggatgggaaggaatgattgcaggttggcacggatacacatcccatggggcacatggagtagcggtggcagcagaccttaagagcactcaagaggccataaacaagataacaaaaaatctcaactctttgagtgagctggaagtaaagaatcttcaaagactaagcggtgccatggatgaactccacaacgaaatactagaactagatgagaaagtggatgatctcagagctgatacaataagctcacaaatagaactcgcagtcctgctttccaatgaaggaataataaacagtgaagatgaacatctcttggcgcttgaaagaaagctgaagaaaatgctgggcccctctgctgtagagatagggaatggatgctttgaaaccaaacacaagtgcaaccagacctgtctcgacagaatagctgctggtacctttgatgcaggagaattttctctccccacctttgattcactgaatattactgctgcatctttaaatgacgatggattggataattaccaaatactgtcaatttattcaacagtggcgagttccctagcactggcaatcatgatggctggtctatctttatggatgtgctccaatggatcgttacaatgcagaatttgcatttaaaggcctattttctttagtttgaatttactgttattcggtgtgcatttctatgtttggtgagcggttttctgtgctcagagtgtgtttattttatgtaatttaatttctttgtgagctcctgtttagcaggtcgtcccttcagcaaggacacaaaaagattttaattttattaaaaaaaaaaaaaaaaaagaccgggaattcgatatcaagcttatcgacctgcagatcgttcaaacatttggcaataaagtttcttaagattgaatcctgttgccggtcttgcgatgattatcatataatttctgttgaattacgttaagcatgtaataattaacatgtaatgcatgacgttatttatgagatgggtttttatgattagagtcccgcaattatacatttaatacgcgatagaaaacaaaatatagcgcgcaaactaggataaattatcgcgcgcggtgtcatctatgttactagatctctagagtctcaagcttggcgcggggtaccgagctcgaattccgagtgtacttcaagtcagttggaaatcaataaaatgattattttatgaatatatttcattgtgcaagtagatagaaattacatatgttacataacacacgaaataaacaaaaaaacacaatccaaaacaaacaccccaaacaaaataacactatatatatcctcgtatgaggagaggcacgttcagtgactcgacgattcccgagcaaaaaaagtctccccgtcacacatatagtgggtgacgcaattatcttcaaagtaatccttctgttgacttgtcattgataacatccagtcttcgtcaggattgcaaagaattatagaagggatcccaccttttattttcttcttttttccatatttagggttgacagtgaaatcagactggcaacctattaattgcttccacaatgggacgaacttgaaggggatgtcgtcgatgatattataggtggcgtgttcatcgtagttggtgaagtcgatggtcccgttccagtagttgtgtcgcccgagacttctagcccaggtggtctttccggtacgagttggtccgcagatgtagaggctggggtgtctgaccccagtccttccctcatcctggttagatcggccatccactcaaggtcagattgtgcttgatcgtaggagacaggatgtatgaaagtgtaggcatcgatgcttacatgatataggtgcgtctctctccagttgtgcagatcttcgtggcagcggagatctgattctgtgaagggcgacacgtactgctcaggttgtggaggaaataatttgttggctgaatattccagccattgaagctttgttgcccattcatgagggaattcttctttgatcatgtcaagatactcctccttagacgttgcagtctggataatagttcgccatcgtgcgtcagatttgcgaggagagaccttatgatctcggaaatctcctctggttttaatatctccgtcctttgatatgtaatcaaggacttgtttagagtttctagctggctggatattagggtgatttccttcaaaatcgaaaaaagaaggatccctaatacaaggttttttatcaagctggataagagcatgatagtgggtagtgccatcttgatgaagctcagaagcaacaccaaggaagaaaataagaaaaggtgtgagtttctcccagagaaactggaataaatcatctctttgagatgagcacttggggtaggtaaggaaaacatatttagattggagtctgaagttcttgctagcagaaggcatgttgttgtgactccgaggggttgcctcaaactctatcttataaccggcgtggaggcatggaggcaagggcattttggtaatttaagtagttagtggaaaatgacgtcatttacttaaagacgaagtcttgcgacaaggggggcccacgccgaattttaatattaccggcgtggccccaccttatcgcgagtgctttagcacgagcggtccagatttaaagtagaaaagttcccgcccactagggttaaaggtgttcacactataaaagcatatacgatgtgatggtatttgatggagcgtatattgtatcaggtatttccgtcggatacgaattattcgtac

SEQ ID NO: 37 - protein, 594 aa, Influenza virus
MAKNVAIFGLLFSLLVLVPSQIFADRICTGITSSNSPHVVKTATQGEVNVTGVIPLTTTPTKSHFANLKGTETRGKLCPKCLNCTDLDVALGRPKCTGKIPSARVSILHEVRPVTSGCFPIMHDRTKIRQLPNLLRGYEHIRLSTHNVINAENAPGGPYKIGTSGSCPNITNGNGFFATMAWAVPKNDKNKTATNPLTIEVPYICTEGEDQITVWGFHSDNETQMAKLYGDSKPQKFTSSANGVTTHYVSQIGGFPNQTEDGGLPQSGRIVVDYMVQKSGKTGTITYQRGILLPQKVWCASGRSKVIKGSLPLIGEADCLHEKYGGLNKSKPYYTGEHAKAIGNCPIWVKTPLKLANGTKYRPPAKLLKERGFFGAIAGFLEGGWEGMIAGWHGYTSHGAHGVAVAADLKSTQEAINKITKNLNSLSELEVKNLQRLSGAMDELHNEILELDEKVDDLRADTISSQIELAVLLSNEGIINSEDEHLLALERKLKKMLGPSAVEIGNGCFETKHKCNQTCLDRIAAGTFDAGEFSLPTFDSLNITAASLNDDGLDNYQILSIYSTVASSLALAIMMAGLSLWMCSNGSLQCRICI

SEQ ID NO: 38 - DNA, 52 bp, Artificial Sequence
  primer 1039+1059.r
cttcccatcctccaccaggaggtctatatttggttccattggccagcttcaa

SEQ ID NO: 39 - DNA, 52 bp, Artificial Sequence
  primer 1039+1059.c
caaatatagacctcctggtggaggatgggaaggaatgattgcaggttggcac

SEQ ID NO: 40 - DNA, 5504 bp, Artificial Sequence
  Expression cassette number 1059 from BeYDV left LIR to BeYDV right LIR. PDISP/HA from influenza B/Brisbane/60/2008 with deleted proteolytic loop
ctagcagaaggcatgttgttgtgactccgaggggttgcctcaaactctatcttataaccggcgtggaggcatggaggcaagggcattttggtaatttaagtagttagtggaaaatgacgtcatttacttaaagacgaagtcttgcgacaaggggggcccacgccgaattttaatattaccggcgtggccccaccttatcgcgagtgctttagcacgagcggtccagatttaaagtagaaaagttcccgcccactagggttaaaggtgttcacactataaaagcatatacgatgtgatggtatttgataaagcgtatattgtatcaggtatttccgtcggatacgaattattcgtacaagcttcttaagccggtcaacatggtggagcacgacacacttgtctactccaaaaatatcaaagatacagtctcagaagaccaaagggcaattgagacttttcaacaaagggtaatatccggaaacctcctcggattccattgcccagctatctgtcactttattgtgaagatagtggaaaaggaaggtggctcctacaaatgccatcattgcgataaaggaaaggccatcgttgaagatgcctctgccgacagtggtcccaaagatggacccccacccacgaggagcatcgtggaaaaagaagacgttccaaccacgtcttcaaagcaagtggattgatgtgataacatggtggagcacgacacacttgtctactccaaaaatatcaaagatacagtctcagaagaccaaagggcaattgagacttttcaacaaagggtaatatccggaaacctcctcggattccattgcccagctatctgtcactttattgtgaagatagtggaaaaggaaggtggctcctacaaatgccatcattgcgataaaggaaaggccatcgttgaagatgcctctgccgacagtggtcccaaagatggacccccacccacgaggagcatcgtggaaaaagaagacgttccaaccacgtcttcaaagcaagtggattgatgtgatatctccactgacgtaagggatgacgcacaatcccactatccttcgcaagacccttcctctatataaggaagttcatttcatttggagaggtattaaaatcttaataggttttgataaaagcgaacgtggggaaacccgaaccaaaccttcttctaaactctctctcatctctcttaaagcaaacttctctcttgtctttcttgcgtgagcgatcttcaacgttgtcagatcgtgcttcggcaccagtacaacgttttctttcactgaagcgaaatcaaagatctctttgtggacacgtagtgcggcgccattaaataacgtgtacttgtcctattcttgtcggtgtggtcttgggaaaagaaagcttgctggaggctgctgttcagccccatacattacttgttacgattctgctgactttcggcgggtgcaatatctctacttctgcttgacgaggtattgttgcctgtacttctttcttcttcttcttgctgattggttctataagaaatctagtattttctttgaaacagagttttcccgtggttttcgaacttggagaaagattgttaagcttctgtatattctgcccaaatttgtcgggcccatggcgaaaaacgttgcgattttcggcttattgttttctcttcttgtgttggttccttctcagatcttcgccgatcgaatctgcactggaataacatcgtcaaactcaccacatgtcgtcaaaactgctactcaaggggaggtcaatgtgactggtgtaataccactgacaacaacacccaccaaatctcattttgcaaatctcaaaggaacagaaaccagggggaaactatgcccaaaatgcctcaactgcacagatctggacgtagccttgggcagaccaaaatgcacggggaaaataccctcggcaagagtttcaatactccatgaagtcagacctgttacatctgggtgctttcctataatgcacgacagaacaaaaattagacagctgcctaaccttctccgaggatacgaacatatcaggttatcaacccataacgttatcaatgcagaaaatgcaccaggaggaccctacaaaattggaacctcagggtcttgccctaacattaccaatggaaacggatttttcgcaacaatggcttgggccgtcccaaaaaacgacaaaaacaaaacagcaacaaatccattaacaatagaagtaccatacatttgtacagaaggagaagaccaaattaccgtttgggggttccactctgacaacgagacccaaatggcaaagctctatggggactcaaagccccagaagttcacctcatctgccaacggagtgaccacacattacgtttcacagattggtggcttcccaaatcaaacagaagacggaggactaccacaaagtggtagaattgttgttgattacatggtgcaaaaatctgggaaaacaggaacaattacctatcaaaggggtattttattgcctcaaaaggtgtggtgcgcaagtggcaggagcaaggtaataaaaggatccttgcctttaattggagaagcagattgcctccacgaaaaatacggtggattaaacaaaagcaagccttactacacaggggaacatgcaaaggccataggaaattgcccaatatgggtgaaaacacccttgaagctggccaatggaaccaaatatagacctcctggtggaggatgggaaggaatgattgcaggttggcacggatacacatcccatggggcacatggagtagcggtggcagcagaccttaagagcactcaagaggccataaacaagataacaaaaaatctcaactctttgagtgagctggaagtaaagaatcttcaaagactaagcggtgccatggatgaactccacaacgaaatactagaactagatgagaaagtggatgatctcagagctgatacaataagctcacaaatagaactcgcagtcctgctttccaatgaaggaataataaacagtgaagatgaacatctcttggcgcttgaaagaaagctgaagaaaatgctgggcccctctgctgtagagatagggaatggatgctttgaaaccaaacacaagtgcaaccagacctgtctcgacagaatagctgctggtacctttgatgcaggagaattttctctccccacctttgattcactgaatattactgctgcatctttaaatgacgatggattggataatcatactatactgctttactactcaactgctgcctccagtttggctgtaacactgatgatagctatctttgttgtttatatggtctccagagacaatgtttcttgctccatctgtctataaaggcctattttctttagtttgaatttactgttattcggtgtgcatttctatgtttggtgagcggttttctgtgctcagagtgtgtttattttatgtaatttaatttctttgtgagctcctgtttagcaggtcgtcccttcagcaaggacacaaaaagattttaattttattaaaaaaaaaaaaaaaaaagaccgggaattcgatatcaagcttatcgacctgcagatcgttcaaacatttggcaataaagtttcttaagattgaatcctgttgccggtcttgcgatgattatcatataatttctgttgaattacgttaagcatgtaataattaacatgtaatgcatgacgttatttatgagatgggtttttatgattagagtcccgcaattatacatttaatacgcgatagaaaacaaaatatagcgcgcaaactaggataaattatcgcgcgcggtgtcatctatgttactagatctctagagtctcaagcttggcgcggggtaccgagctcgaattccgagtgtacttcaagtcagttggaaatcaataaaatgattattttatgaatatatttcattgtgcaagtagatagaaattacatatgttacataacacacgaaataaacaaaaaaacacaatccaaaacaaacaccccaaacaaaataacactatatatatcctcgtatgaggagaggcacgttcagtgactcgacgattcccgagcaaaaaaagtctccccgtcacacatatagtgggtgacgcaattatcttcaaagtaatccttctgttgacttgtcattgataacatccagtcttcgtcaggattgcaaagaattatagaagggatcccaccttttattttcttcttttttccatatttagggttgacagtgaaatcagactggcaacctattaattgcttccacaatgggacgaacttgaaggggatgtcgtcgatgatattataggtggcgtgttcatcgtagttggtgaagtcgatggtcccgttccagtagttgtgtcgcccgagacttctagcccaggtggtctttccggtacgagttggtccgcagatgtagaggctggggtgtctgaccccagtccttccctcatcctggttagatcggccatccactcaaggtcagattgtgcttgatcgtaggagacaggatgtatgaaagtgtaggcatcgatgcttacatgatataggtgcgtctctctccagttgtgcagatcttcgtggcagcggagatctgattctgtgaagggcgacacgtactgctcaggttgtggaggaaataatttgttggctgaatattccagccattgaagctttgttgcccattcatgagggaattcttctttgatcatgtcaagatactcctccttagacgttgcagtctggataatagttcgccatcgtgcgtcagatttgcgaggagagaccttatgatctcggaaatctcctctggttttaatatctccgtcctttgatatgtaatcaaggacttgtttagagtttctagctggctggatattagggtgatttccttcaaaatcgaaaaaagaaggatccctaatacaaggttttttatcaagctggataagagcatgatagtgggtagtgccatcttgatgaagctcagaagcaacaccaaggaagaaaataagaaaaggtgtgagtttctcccagagaaactggaataaatcatctctttgagatgagcacttggggtaggtaaggaaaacatatttagattggagtctgaagttcttgctagcagaaggcatgttgttgtgactccgaggggttgcctcaaactctatcttataaccggcgtggaggcatggaggcaagggcattttggtaatttaagtagttagtggaaaatgacgtcatttacttaaagacgaagtcttgcgacaaggggggcccacgccgaattttaatattaccggcgtggccccaccttatcgcgagtgctttagcacgagcggtccagatttaaagtagaaaagttcccgcccactagggttaaaggtgttcacactataaaagcatatacgatgtgatggtatttgatggagcgtatattgtatcaggtatttccgtcggatacgaattattcgtac

SEQ ID NO: 41 - protein, 577 aa, Influenza virus
MAKNVAIFGLLFSLLVLVPSQIFADRICTGITSSNSPHVVKTATQGEVNVTGVIPLTTTPTKSHFANLKGTETRGKLCPKCLNCTDLDVALGRPKCTGKIPSARVSILHEVRPVTSGCFPIMHDRTKIRQLPNLLRGYEHIRLSTHNVINAENAPGGPYKIGTSGSCPNITNGNGFFATMAWAVPKNDKNKTATNPLTIEVPYICTEGEDQITVWGFHSDNETQMAKLYGDSKPQKFTSSANGVTTHYVSQIGGFPNQTEDGGLPQSGRIVVDYMVQKSGKTGTITYQRGILLPQKVWCASGRSKVIKGSLPLIGEADCLHEKYGGLNKSKPYYTGEHAKAIGNCPIWVKTPLKLANGTKYRPPGGGWEGMIAGWHGYTSHGAHGVAVAADLKSTQEAINKITKNLNSLSELEVKNLQRLSGAMDELHNEILELDEKVDDLRADTISSQIELAVLLSNEGIINSEDEHLLALERKLKKMLGPSAVEIGNGCFETKHKCNQTCLDRIAAGTFDAGEFSLPTFDSLNITAASLNDDGLDNHTILLYYSTAASSLAVTLMIAIFVVYMVSRDNVSCSICL

SEQ ID NO: 42 - DNA, 1707 bp, Influenza virus
atggagaaaatagtgcttcttcttgcaatagtcagtcttgttaaaagtgatcagatttgcattggttaccatgcaaacaattcaacagagcaggttgacacaatcatggaaaagaacgttactgttacacatgcccaagacatactggaaaagacacacaacgggaagctctgcgatctagatggagtgaagcctctaattttaagagattgtagtgtagctggatggctcctcgggaacccaatgtgtgacgaattcatcaatgtaccggaatggtcttacatagtggagaaggccaatccaaccaatgacctctgttacccagggagtttcaacgactatgaagaactgaaacacctattgagcagaataaaccattttgagaaaattcaaatcatccccaaaagttcttggtccgatcatgaagcctcatcaggagttagctcagcatgtccatacctgggaagtccctccttttttagaaatgtggtatggcttatcaaaaagaacagtacatacccaacaataaagaaaagctacaataataccaaccaagaggatcttttggtactgtggggaattcaccatcctaatgatgcggcagagcagacaaggctatatcaaaacccaaccacctatatttccattgggacatcaacactaaaccagagattggtaccaaaaatagctactagatccaaagtaaacgggcaaagtggaaggatggagttcttctggacaattttaaaacctaatgatgcaatcaacttcgagagtaatggaaatttcattgctccagaatatgcatacaaaattgtcaagaaaggggactcagcaattatgaaaagtgaattggaatatggtaactgcaacaccaagtgtcaaactccaatgggggcgataaactctagtatgccattccacaacatacaccctctcaccatcggggaatgccccaaatatgtgaaatcaaacagattagtccttgcaacagggctcagaaatagccctcaaagagagagcagaagaaaaaagagaggactatttggagctatagcaggttttatagagggaggatggcagggaatggtagatggttggtatgggtaccaccatagcaatgagcaggggagtgggtacgctgcagacaaagaatccactcaaaaggcaatagatggagtcaccaataaggtcaactcaatcattgacaaaatgaacactcagtttgaggccgttggaagggaatttaataacttagaaaggagaatagagaatttaaacaagaagatggaagacgggtttctagatgtctggacttataatgccgaacttctggttctcatggaaaatgagagaactctagactttcatgactcaaatgttaagaacctctacgacaaggtccgactacagcttagggataatgcaaaggagctgggtaacggttgtttcgagttctatcacaaatgtgataatgaatgtatggaaagtataagaaacggaacgtacaactatccgcagtattcagaagaagcaagattaaaaagagaggaaataagtggggtaaaattggaatcaataggaacttaccaaatactgtcaatttattcaacagtggcgagttccctagcactggcaatcatgatggctggtctatctttatggatgtgctccaatggatcgttacaatgcagaatttgcatttaa

SEQ ID NO: 43 - DNA, 1734 bp, Influenza virus
atggcgaaaaacgttgcgattttcggcttattgttttctcttcttgtgttggttccttctcagatcttcgccgatcgaatctgcactggaataacatcgtcaaactcaccacatgtcgtcaaaactgctactcaaggggaggtcaatgtgactggtgtaataccactgacaacaacacccaccaaatctcattttgcaaatctcaaaggaacagaaaccagggggaaactatgcccaaaatgcctcaactgcacagatctggacgtagccttgggcagaccaaaatgcacggggaaaataccctcggcaagagtttcaatactccatgaagtcagacctgttacatctgggtgctttcctataatgcacgacagaacaaaaattagacagctgcctaaccttctccgaggatacgaacatatcaggttatcaacccataacgttatcaatgcagaaaatgcaccaggaggaccctacaaaattggaacctcagggtcttgccctaacattaccaatggaaacggatttttcgcaacaatggcttgggccgtcccaaaaaacgacaaaaacaaaacagcaacaaatccattaacaatagaagtaccatacatttgtacagaaggagaagaccaaattaccgtttgggggttccactctgacaacgagacccaaatggcaaagctctatggggactcaaagccccagaagttcacctcatctgccaacggagtgaccacacattacgtttcacagattggtggcttcccaaatcaaacagaagacggaggactaccacaaagtggtagaattgttgttgattacatggtgcaaaaatctgggaaaacaggaacaattacctatcaaaggggtattttattgcctcaaaaggtgtggtgcgcaagtggcaggagcaaggtaataaaaggatccttgcctttaattggagaagcagattgcctccacgaaaaatacggtggattaaacaaaagcaagccttactacacaggggaacatgcaaaggccataggaaattgcccaatatgggtgaaaacacccttgaagctggccaatggaaccaaatatagacctcctggtggaggatgggaaggaatgattgcaggttggcacggatacacatcccatggggcacatggagtagcggtggcagcagaccttaagagcactcaagaggccataaacaagataacaaaaaatctcaactctttgagtgagctggaagtaaagaatcttcaaagactaagcggtgccatggatgaactccacaacgaaatactagaactagatgagaaagtggatgatctcagagctgatacaataagctcacaaatagaactcgcagtcctgctttccaatgaaggaataataaacagtgaagatgaacatctcttggcgcttgaaagaaagctgaagaaaatgctgggcccctctgctgtagagatagggaatggatgctttgaaaccaaacacaagtgcaaccagacctgtctcgacagaatagctgctggtacctttgatgcaggagaattttctctccccacctttgattcactgaatattactgctgcatctttaaatgacgatggattggataatcatactatactgctttactactcaactgctgcctccagtttggctgtaacactgatgatagctatctttgttgtttatatggtctccagagacaatgtttcttgctccatctgtctataa

SEQ ID NO: 44 - DNA, 48 bp, Artificial Sequence
  primer IF-H3V36111.S2+4c
tctcagatcttcgcccaaaaacttcctggaaatgacaacagcacggca

SEQ ID NO: 45 - DNA, 51 bp, Artificial Sequence
  primer IF-H3V36111.s1-4r
actaaagaaaataggccttcaaatgcaaatgttgcacctaatgttgccctt

SEQ ID NO: 46 - DNA, 1701 bp, Artificial Sequence
  nucleotide sequence of synthesized H3 gene
atgaagactatcattgctttgagccacattctatgtctggttttcgctcaaaaacttcctggaaatgacaacagcacggcaacgctgtgccttgggcaccatgcagtaccaaacggaacgatagtgaaaacaatcacgaatgaccaaattgaagttactaatgctactgagctggttcagaattcctcaataggtgaaatatgcgacagtcctcatcagatccttgatggagaaaactgcacactaatagatgctctattgggagaccctcagtgtgatggcttccaaaataagaaatgggacctttttgttgaacgaagcaaagcctacagcaactgttacccttatgatgtgccggattatgcctcccttaggtcactagttgcctcatccggcacactggagtttaacaatgaaagcttcaattggactggagtcactcaaaacggaacaagttctgcttgcataaggagatctaataatagtttctttagtagattaaattggttgacccacttaaacttcaaatacccagcattgaacgtgactatgccaaacaatgaacaatttgacaaattgtacatttggggggttcaccacccgggtacggacaaggaccaaatcttcctgtatgctcaatcatcaggaagaatcacagtatctaccaaaagaagccaacaagctgtaatcccgaatatcggatctagacccagaataaggaatatccctagcagaataagcatctattggacaatagtaaaaccgggagacatacttttgattaacagcacagggaatctaattgctcctaggggttacttcaaaatacgaagtgggaaaagctcaataatgagatcagatgcacccattggcaaatgcaattctgaatgcatcactccaaatggaagcattcccaatgacaaaccattccaaaatgtaaacaggatcacatacggggcctgtcccagatatgttaagcaaagcactctgaaattggcaacaggaatgcgaaatgtaccagagaaacaaactagaggcatatttggcgcaatagcgggtttcatagaaaatggttgggagggaatggtggatggttggtacggtttcaggcatcaaaattctgagggaagaggacaagcagcagatctcaaaagcactcaagcagcaatcgatcaaatcaatgggaagctgaatcgattgatcgggaaaaccaacgagaaattccatcagattgaaaaagaattctcagaagtcgaagggagaattcaggaccttgagaaatatgttgaggacactaaaatagatctctggtcatacaacgcggagcttcttgttgccctggagaaccaacatacaattgatctaactgactcagaaatgaacaaactgtttgaaaaaacaaagaagcaactaagggaaaatgctgaggatatgggcaatggttgtttcaaaatataccacaaatgtgacaatgcctgcataggatcaatcagaaatggaacttatgaccacgatgtatacagagatgaagcattaaacaaccggttccagatcaagggagttgagctgaagtcagggtacaaagattggatcctatggatttcctttgccatatcatgttttttgctttgtgttgctttgttggggttcatcatgtgggcctgccaaaagggcaacattaggtgcaacatttgcatttga

SEQ ID NO: 47 - DNA, 3465 bp, Artificial Sequence
  expression cassette number 1391
gtcaacatggtggagcacgacacacttgtctactccaaaaatatcaaagatacagtctcagaagaccaaagggcaattgagacttttcaacaaagggtaatatccggaaacctcctcggattccattgcccagctatctgtcactttattgtgaagatagtggaaaaggaaggtggctcctacaaatgccatcattgcgataaaggaaaggccatcgttgaagatgcctctgccgacagtggtcccaaagatggacccccacccacgaggagcatcgtggaaaaagaagacgttccaaccacgtcttcaaagcaagtggattgatgtgataacatggtggagcacgacacacttgtctactccaaaaatatcaaagatacagtctcagaagaccaaagggcaattgagacttttcaacaaagggtaatatccggaaacctcctcggattccattgcccagctatctgtcactttattgtgaagatagtggaaaaggaaggtggctcctacaaatgccatcattgcgataaaggaaaggccatcgttgaagatgcctctgccgacagtggtcccaaagatggacccccacccacgaggagcatcgtggaaaaagaagacgttccaaccacgtcttcaaagcaagtggattgatgtgatatctccactgacgtaagggatgacgcacaatcccactatccttcgcaagacccttcctctatataaggaagttcatttcatttggagaggtattaaaatcttaataggttttgataaaagcgaacgtggggaaacccgaaccaaaccttcttctaaactctctctcatctctcttaaagcaaacttctctcttgtctttcttgcgtgagcgatcttcaacgttgtcagatcgtgcttcggcaccagtacaacgttttctttcactgaagcgaaatcaaagatctctttgtggacacgtagtgcggcgccattaaataacgtgtacttgtcctattcttgtcggtgtggtcttgggaaaagaaagcttgctggaggctgctgttcagccccatacattacttgttacgattctgctgactttcggcgggtgcaatatctctacttctgcttgacgaggtattgttgcctgtacttctttcttcttcttcttgctgattggttctataagaaatctagtattttctttgaaacagagttttcccgtggttttcgaacttggagaaagattgttaagcttctgtatattctgcccaaatttgtcgggcccatggcgaaaaacgttgcgattttcggcttattgttttctcttcttgtgttggttccttctcagatcttcgcccaaaaacttcctggaaatgacaacagcacggcaacgctgtgccttgggcaccatgcagtaccaaacggaacgatagtgaaaacaatcacgaatgaccaaattgaagttactaatgctactgagctggttcagaattcctcaataggtgaaatatgcgacagtcctcatcagatccttgatggagaaaactgcacactaatagatgctctattgggagaccctcagtgtgatggcttccaaaataagaaatgggacctttttgttgaacgaagcaaagcctacagcaactgttacccttatgatgtgccggattatgcctcccttaggtcactagttgcctcatccggcacactggagtttaacaatgaaagcttcaattggactggagtcactcaaaacggaacaagttctgcttgcataaggagatctaataatagtttctttagtagattaaattggttgacccacttaaacttcaaatacccagcattgaacgtgactatgccaaacaatgaacaatttgacaaattgtacatttggggggttcaccacccgggtacggacaaggaccaaatcttcctgtatgctcaatcatcaggaagaatcacagtatctaccaaaagaagccaacaagctgtaatcccgaatatcggatctagacccagaataaggaatatccctagcagaataagcatctattggacaatagtaaaaccgggagacatacttttgattaacagcacagggaatctaattgctcctaggggttacttcaaaatacgaagtgggaaaagctcaataatgagatcagatgcacccattggcaaatgcaattctgaatgcatcactccaaatggaagcattcccaatgacaaaccattccaaaatgtaaacaggatcacatacggggcctgtcccagatatgttaagcaaagcactctgaaattggcaacaggaatgcgaaatgtaccagagaaacaaactagaggcatatttggcgcaatagcgggtttcatagaaaatggttgggagggaatggtggatggttggtacggtttcaggcatcaaaattctgagggaagaggacaagcagcagatctcaaaagcactcaagcagcaatcgatcaaatcaatgggaagctgaatcgattgatcgggaaaaccaacgagaaattccatcagattgaaaaagaattctcagaagtcgaagggagaattcaggaccttgagaaatatgttgaggacactaaaatagatctctggtcatacaacgcggagcttcttgttgccctggagaaccaacatacaattgatctaactgactcagaaatgaacaaactgtttgaaaaaacaaagaagcaactaagggaaaatgctgaggatatgggcaatggttgtttcaaaatataccacaaatgtgacaatgcctgcataggatcaatcagaaatggaacttatgaccacgatgtatacagagatgaagcattaaacaaccggttccagatcaagggagttgagctgaagtcagggtacaaagattggatcctatggatttcctttgccatatcatgttttttgctttgtgttgctttgttggggttcatcatgtgggcctgccaaaagggcaacattaggtgcaacatttgcatttgaaggcctattttctttagtttgaatttactgttattcggtgtgcatttctatgtttggtgagcggttttctgtgctcagagtgtgtttattttatgtaatttaatttctttgtgagctcctgtttagcaggtcgtcccttcagcaaggacacaaaaagattttaattttattaaaaaaaaaaaaaaaaaagaccgggaattcgatatcaagcttatcgacctgcagatcgttcaaacatttggcaataaagtttcttaagattgaatcctgttgccggtcttgcgatgattatcatataatttctgttgaattacgttaagcatgtaataattaacatgtaatgcatgacgttatttatgagatgggtttttatgattagagtcccgcaattatacatttaatacgcgatagaaaacaaaatatagcgcgcaaactaggataaattatcgcgcgcggtgtcatctatgttactagat

SEQ ID NO: 48 - protein, 574 aa, Influenza virus
MAKNVAIFGLLFSLLVLVPSQIFAQKLPGNDNSTATLCLGHHAVPNGTIVKTITNDQIEVTNATELVQNSSIGEICDSPHQILDGENCTLIDALLGDPQCDGFQNKKWDLFVERSKAYSNCYPYDVPDYASLRSLVASSGTLEFNNESFNWTGVTQNGTSSACIRRSNNSFFSRLNWLTHLNFKYPALNVTMPNNEQFDKLYIWGVHHPGTDKDQIFLYAQSSGRITVSTKRSQQAVIPNIGSRPRIRNIPSRISIYWTIVKPGDILLINSTGNLIAPRGYFKIRSGKSSIMRSDAPIGKCNSECITPNGSIPNDKPFQNVNRITYGACPRYVKQSTLKLATGMRNVPEKQTRGIFGAIAGFIENGWEGMVDGWYGFRHQNSEGRGQAADLKSTQAAIDQINGKLNRLIGKTNEKFHQIEKEFSEVEGRIQDLEKYVEDTKIDLWSYNAELLVALENQHTIDLTDSEMNKLFEKTKKQLRENAEDMGNGCFKIYHKCDNACIGSIRNGTYDHDVYRDEALNNRFQIKGVELKSGYKDWILWISFAISCFLLCVALLGFIMWACQKGNIRCNICI

SEQ ID NO: 49 - DNA, 46 bp, Artificial Sequence
  primer IF-HAB110.S1+3c
aaatttgtcgggcccatgaaggcaataattgtactactcatggtag

SEQ ID NO: 50 - DNA, 52 bp, Artificial Sequence
  primer IF-HAB110.s1-4r
actaaagaaaataggcctttatagacagatggagcatgaaacgttgtctctg

SEQ ID NO: 51 - DNA, 1755 bp, Artificial Sequence
  nucleotide sequence of synthesized HA B/Wisconin (JN993010)
atgaaggcaataattgtactactcatggtagtaacatccaatgcagatcgaatctgcactgggataacatcttcaaactcacctcatgtggtcaaaacagctactcaaggggaggtcaatgtgactggcgtgataccactgacaacaacaccaacaaaatcttattttgcaaatctcaaaggaacaaggaccagagggaaactatgcccggactgtctcaactgtacagatctggatgtggccttgggcaggccaatgtgtgtggggaccacaccttctgctaaagcttcaatactccacgaggtcagacctgttacatccgggtgctttcctataatgcacgacagaacaaaaatcaggcaactacccaatcttctcagaggatatgaaaatatcaggttatcaacccaaaacgttatcgatgcagaaaaagcaccaggaggaccctacagacttggaacctcaggatcttgccctaacgctaccagtaaaatcggattttttgcaacaatggcttgggctgtcccaaaggacaactacaaaaatgcaacgaacccactaacagtagaagtaccatacatttgtacagaaggggaagaccaaattactgtttgggggttccattcagataacaaaacccaaatgaagagcctctatggagactcaaatcctcaaaagttcacctcatctgctaatggagtaaccacacattatgtttctcagattggcgacttcccagatcaaacagaagacggaggactaccacaaagcggcagaattgttgttgattacatgatgcaaaaacctgggaaaacaggaacaattgtctatcaaagaggtgttttgttgcctcaaaaggtgtggtgcgcgagtggcaggagcaaagtaataaaagggtcattgcctttaattggtgaagcagattgccttcatgaaaaatacggtggattaaacaaaagcaagccttactacacaggagaacatgcaaaagccataggaaattgcccaatatgggtaaaaacacctttgaagcttgccaatggaaccaaatatagacctcctgcaaaactattgaaggaaaggggtttcttcggagctattgctggtttcctagaaggaggatgggaaggaatgattgcaggttggcacggatacacatctcacggagcacatggagtggcagtggcggcagaccttaagagtacacaagaagctataaataagataacaaaaaatctcaattctttgagtgagctagaagtaaagaaccttcaaagactaagtggtgccatggatgaactccacaacgaaatactcgagctggatgagaaagtggatgatctcagagctgacactataagctcacaaatagaacttgcagtcttgctttccaacgaaggaataataaacagtgaagacgagcatctattggcacttgagagaaaactaaagaaaatgctgggtccctctgctgtagacataggaaacggatgcttcgaaaccaaacacaaatgcaaccagacctgcttagacaggatagctgctggcacctttaatgcaggagaattttctctccccacttttgattcattgaacattactgctgcatctttaaatgatgatggattggataaccatactatactgctctattactcaactgctgcttctagtttggctgtaacattaatgctagctatttttattgtttatatggtctccagagacaacgtttcatgctccatctgtctataa

SEQ ID NO: 52 - DNA, 6745 bp, Artificial Sequence
  Construct 193
tggcaggatatattgtggtgtaaacaaattgacgcttagacaacttaataacacattgcggacgtttttaatgtactgaattaacgccgaatcccgggctggtatatttatatgttgtcaaataactcaaaaaccataaaagtttaagttagcaagtgtgtacatttttacttgaacaaaaatattcacctactactgttataaatcattattaaacattagagtaaagaaatatggatgataagaacaagagtagtgatattttgacaacaattttgttgcaacatttgagaaaattttgttgttctctcttttcattggtcaaaaacaatagagagagaaaaaggaagagggagaataaaaacataatgtgagtatgagagagaaagttgtacaaaagttgtaccaaaatagttgtacaaatatcattgaggaatttgacaaaagctacacaaataagggttaattgctgtaaataaataaggatgacgcattagagagatgtaccattagagaatttttggcaagtcattaaaaagaaagaataaattatttttaaaattaaaagttgagtcatttgattaaacatgtgattatttaatgaattgatgaaagagttggattaaagttgtattagtaattagaatttggtgtcaaatttaatttgacatttgatcttttcctatatattgccccatagagtcagttaactcatttttatatttcatagatcaaataagagaaataacggtatattaatccctccaaaaaaaaaaaacggtatatttactaaaaaatctaagccacgtaggaggataacaggatccccgtaggaggataacatccaatccaaccaatcacaacaatcctgatgagataacccactttaagcccacgcatctgtggcacatctacattatctaaatcacacattcttccacacatctgagccacacaaaaaccaatccacatctttatcacccattctataaaaaatcacactttgtgagtctacactttgattcccttcaaacacatacaaagagaagagactaattaattaattaatcatcttgagagaaaatggaacgagctatacaaggaaacgacgctagggaacaagctaacagtgaacgttgggatggaggatcaggaggtaccacttctcccttcaaacttcctgacgaaagtccgagttggactgagtggcggctacataacgatgagacgaattcgaatcaagataatccccttggtttcaaggaaagctggggtttcgggaaagttgtatttaagagatatctcagatacgacaggacggaagcttcactgcacagagtccttggatcttggacgggagattcggttaactatgcagcatctcgatttttcggtttcgaccagatcggatgtacctatagtattcggtttcgaggagttagtatcaccgtttctggagggtcgcgaactcttcagcatctctgtgagatggcaattcggtctaagcaagaactgctacagcttgccccaatcgaagtggaaagtaatgtatcaagaggatgccctgaaggtactcaaaccttcgaaaaagaaagcgagtaagttaaaatgcttcttcgtctcctatttataatatggtttgttattgttaattttgttcttgtagaagagcttaattaatcgttgttgttatgaaatactatttgtatgagatgaactggtgtaatgtaattcatttacataagtggagtcagaatcagaatgtttcctccataactaactagacatgaagacctgccgcgtacaattgtcttatatttgaacaactaaaattgaacatcttttgccacaactttataagtggttaatatagctcaaatatatggtcaagttcaatagattaataatggaaatatcagttatcgaaattcattaacaatcaacttaacgttattaactactaattttatatcatcccctttgataaatgatagtacaccaattaggaaggagcatgctcgcctaggagattgtcgtttcccgccttcagtttgcaagctgctctagccgtgtagccaatacgcaaaccgcctctccccgcgcgttgggaattactagcgcgtgtcgagacgcgttgttgttgtgactccgaggggttgcctcaaactctatcttataaccggcgtggaggcatggaggcaggggtattttggtcattttaatagatagtggaaaatgacgtggaatttacttaaagacgaagtctttgcgacaagggggggcccacgccgaatttaatattaccggcgtggcccccccttatcgcgagtgctttagcacgagcggtccagatttaaagtagaaaatttcccgcccactagggttaaaggtgttcacactataaaagcatatacgatgtgatggtatttggtcgacaagcttgcatgccggtcaacatggtggagcacgacacacttgtctactccaaaaatatcaaagatacagtctcagaagaccaaagggcaattgagacttttcaacaaagggtaatatccggaaacctcctcggattccattgcccagctatctgtcactttattgtgaagatagtggaaaaggaaggtggctcctacaaatgccatcattgcgataaaggaaaggccatcgttgaagatgcctctgccgacagtggtcccaaagatggacccccacccacgaggagcatcgtggaaaaagaagacgttccaaccacgtcttcaaagcaagtggattgatgtgataacatggtggagcacgacacacttgtctactccaaaaatatcaaagatacagtctcagaagaccaaagggcaattgagacttttcaacaaagggtaatatccggaaacctcctcggattccattgcccagctatctgtcactttattgtgaagatagtggaaaaggaaggtggctcctacaaatgccatcattgcgataaaggaaaggccatcgttgaagatgcctctgccgacagtggtcccaaagatggacccccacccacgaggagcatcgtggaaaaagaagacgttccaaccacgtcttcaaagcaagtggattgatgtgatatctccactgacgtaagggatgacgcacaatcccactatccttcgcaagacccttcctctatataaggaagttcatttcatttggagaggtattaaaatcttaataggttttgataaaagcgaacgtggggaaacccgaaccaaaccttcttctaaactctctctcatctctcttaaagcaaacttctctcttgtctttcttgcgtgagcgatcttcaacgttgtcagatcgtgcttcggcaccagtacaacgttttctttcactgaagcgaaatcaaagatctctttgtggacacgtagtgcggcgccattaaataacgtgtacttgtcctattcttgtcggtgtggtcttgggaaaagaaagcttgctggaggctgctgttcagccccatacattacttgttacgattctgctgactttcggcgggtgcaatatctctacttctgcttgacgaggtattgttgcctgtacttctttcttcttcttcttgctgattggttctataagaaatctagtattttctttgaaacagagttttcccgtggttttcgaacttggagaaagattgttaagcttctgtatattctgcccaaatttgtcgggcccgcggatggcgaaaaacgttgcgattttcggcttattgttttctcttcttgtgttggttccttctcagatcttcgcctgcaggctcctcagccaaaacgacacccccatctgtctatccactggcccctggatctgctgcccaaactaactccatggtgaccctgggatgcctggtcaagggctatttccctgagccagtgacagtgacctggaactctggatccctgtccagcggtgtgcacaccttcccagctgtcctgcagtctgacctctacactctgagcagctcagtgactgtcccctccagcacctggcccagcgagaccgtcacctgcaacgttgcccacccggccagcagcaccaaggtggacaagaaaattgtgcccagggattgtggttgtaagccttgcatatgtacagtcccagaagtatcatctgtcttcatcttccccccaaagcccaaggatgtgctcaccattactctgactcctaaggtcacgtgtgttgtggtagacatcagcaaggatgatcccgaggtccagttcagctggtttgtagatgatgtggaggtgcacacagctcagacgcaaccccgggaggagcagttcaacagcactttccgctcagtcagtgaacttcccatcatgcaccaggactggctcaatggcaaggagcgatcgctcaccatcaccatcaccatcaccatcaccattaaaggcctattttctttagtttgaatttactgttattcggtgtgcatttctatgtttggtgagcggttttctgtgctcagagtgtgtttattttatgtaatttaatttctttgtgagctcctgtttagcaggtcgtcccttcagcaaggacacaaaaagattttaattttattaaaaaaaaaaaaaaaaaagaccgggaattcgatatcaagcttatcgacctgcagatcgttcaaacatttggcaataaagtttcttaagattgaatcctgttgccggtcttgcgatgattatcatataatttctgttgaattacgttaagcatgtaataattaacatgtaatgcatgacgttatttatgagatgggtttttatgattagagtcccgcaattatacatttaatacgcgatagaaaacaaaatatagcgcgcaaactaggataaattatcgcgcgcggtgtcatctatgttactagatctctagagtctcaagcttggcgcgccataaaatgattattttatgaatatatttcattgtgcaagtagatagaaattacatatgttacataacacacgaaataaacaaaaaaagacaatccaaaaacaaacaccccaaaaaaaataatcactttagataaactcgtatgaggagaggcacgttcagtgactcgacgattcccgagcaaaaaaagtctccccgtcacacatatagtgggtgacgcaattatctttaaagtaatccttctgttgacttgtcattgataacatccagtcttcgtcaggattgcaaagaattatagaagggatcccaccttttattttcttcttttttccatatttagggttgacagtgaaatcagactggcaacctattaattgcttccacaatgggacgaacttgaaggggatgtcgtcgatgatattataggtggcgtgttcatcgtagttggtgaaatcgatggtaccgttccaatagttgtgtcgtccgagacttctagcccaggtggtctttccggtacgagttggtccgcagatgtagaggctggggtgtcggattccattccttccattgtcctggttaaatcggccatccattcaaggtcagattgagcttgttggtatgagacaggatgtatgtaagtataagcgtctatgcttacatggtatagatgggtttccctccaggagtgtagatcttcgtggcagcgaagatctgattctgtgaagggcgacacatacggttcaggttgtggagggaataatttgttggctgaatattccagccattgaagttttgttgcccattcatgagggaattcttccttgatcatgtcaagatattcctccttagacgttgcagtctggataatagttctccatcgtgcgtcagatttgcgaggagagaccttatgatctcggaaatctcctctggttttaatatctccgtcctttgatatgtaatcaaggacttgtttagagtttctagctggctggatattagggtgatttccttcaaaatcgaaaaaagaaggatccctaatacaaggttttttatcaagctggagaagagcatgatagtgggtagtgccatcttgatgaagctcagaagcaacaccaaggaagaaaataagaaaaggtgtgagtttctcccagagaaactggaataaatcatctctttgagatgagcacttgggataggtaaggaaaacatatttagattggagtctgaagttcttactagcagaaggcatgttgttgtgactccgaggggttgcctcaaactctatcttataaccggcgtggaggcatggaggcaggggtattttggtcattttaatagatagtggaaaatgacgtggaatttacttaaagacgaagtctttgcgacaagggggggcccacgccgaatttaatattaccggcgtggcccccccttatcgcgagtgctttagcacgagcggtccagatttaaagtagaaaatttcccgcccactagggttaaaggtgttcacactataaaagcatatacgatgtgatggtatttgactagtggcactggccgtcgttttacaacgtcgtgactgggaaaaccctggcgttacccaacttaatcgccttgcagcacatccccctttcgccagctggcgtaatagcgaagaggcccgcaccgatcgcccttcccaacagttgcgcagcctgaatggcgaatgctagagcagcttgagcttggatcagattgtcgtttcccgccttcagtttaaactatcagtgtttgacaggatatattggcgggtaaacctaagagaaaagagcgttta

SEQ ID NO: 53 - DNA, 3495 bp, Artificial Sequence
  Expression cassette number 1462
gtcaacatggtggagcacgacacacttgtctactccaaaaatatcaaagatacagtctcagaagaccaaagggcaattgagacttttcaacaaagggtaatatccggaaacctcctcggattccattgcccagctatctgtcactttattgtgaagatagtggaaaaggaaggtggctcctacaaatgccatcattgcgataaaggaaaggccatcgttgaagatgcctctgccgacagtggtcccaaagatggacccccacccacgaggagcatcgtggaaaaagaagacgttccaaccacgtcttcaaagcaagtggattgatgtgataacatggtggagcacgacacacttgtctactccaaaaatatcaaagatacagtctcagaagaccaaagggcaattgagacttttcaacaaagggtaatatccggaaacctcctcggattccattgcccagctatctgtcactttattgtgaagatagtggaaaaggaaggtggctcctacaaatgccatcattgcgataaaggaaaggccatcgttgaagatgcctctgccgacagtggtcccaaagatggacccccacccacgaggagcatcgtggaaaaagaagacgttccaaccacgtcttcaaagcaagtggattgatgtgatatctccactgacgtaagggatgacgcacaatcccactatccttcgcaagacccttcctctatataaggaagttcatttcatttggagaggtattaaaatcttaataggttttgataaaagcgaacgtggggaaacccgaaccaaaccttcttctaaactctctctcatctctcttaaagcaaacttctctcttgtctttcttgcgtgagcgatcttcaacgttgtcagatcgtgcttcggcaccagtacaacgttttctttcactgaagcgaaatcaaagatctctttgtggacacgtagtgcggcgccattaaataacgtgtacttgtcctattcttgtcggtgtggtcttgggaaaagaaagcttgctggaggctgctgttcagccccatacattacttgttacgattctgctgactttcggcgggtgcaatatctctacttctgcttgacgaggtattgttgcctgtacttctttcttcttcttcttgctgattggttctataagaaatctagtattttctttgaaacagagttttcccgtggttttcgaacttggagaaagattgttaagcttctgtatattctgcccaaatttgtcgggcccatgaaggcaataattgtactactcatggtagtaacatccaatgcagatcgaatctgcactgggataacatcttcaaactcacctcatgtggtcaaaacagctactcaaggggaggtcaatgtgactggcgtgataccactgacaacaacaccaacaaaatcttattttgcaaatctcaaaggaacaaggaccagagggaaactatgcccggactgtctcaactgtacagatctggatgtggccttgggcaggccaatgtgtgtggggaccacaccttctgctaaagcttcaatactccacgaggtcagacctgttacatccgggtgctttcctataatgcacgacagaacaaaaatcaggcaactacccaatcttctcagaggatatgaaaatatcaggttatcaacccaaaacgttatcgatgcagaaaaagcaccaggaggaccctacagacttggaacctcaggatcttgccctaacgctaccagtaaaatcggattttttgcaacaatggcttgggctgtcccaaaggacaactacaaaaatgcaacgaacccactaacagtagaagtaccatacatttgtacagaaggggaagaccaaattactgtttgggggttccattcagataacaaaacccaaatgaagagcctctatggagactcaaatcctcaaaagttcacctcatctgctaatggagtaaccacacattatgtttctcagattggcgacttcccagatcaaacagaagacggaggactaccacaaagcggcagaattgttgttgattacatgatgcaaaaacctgggaaaacaggaacaattgtctatcaaagaggtgttttgttgcctcaaaaggtgtggtgcgcgagtggcaggagcaaagtaataaaagggtcattgcctttaattggtgaagcagattgccttcatgaaaaatacggtggattaaacaaaagcaagccttactacacaggagaacatgcaaaagccataggaaattgcccaatatgggtaaaaacacctttgaagcttgccaatggaaccaaatatagacctcctgcaaaactattgaaggaaaggggtttcttcggagctattgctggtttcctagaaggaggatgggaaggaatgattgcaggttggcacggatacacatctcacggagcacatggagtggcagtggcggcagaccttaagagtacacaagaagctataaataagataacaaaaaatctcaattctttgagtgagctagaagtaaagaaccttcaaagactaagtggtgccatggatgaactccacaacgaaatactcgagctggatgagaaagtggatgatctcagagctgacactataagctcacaaatagaacttgcagtcttgctttccaacgaaggaataataaacagtgaagacgagcatctattggcacttgagagaaaactaaagaaaatgctgggtccctctgctgtagacataggaaacggatgcttcgaaaccaaacacaaatgcaaccagacctgcttagacaggatagctgctggcacctttaatgcaggagaattttctctccccacttttgattcattgaacattactgctgcatctttaaatgatgatggattggataaccatactatactgctctattactcaactgctgcttctagtttggctgtaacattaatgctagctatttttattgtttatatggtctccagagacaacgtttcatgctccatctgtctataaaggcctattttctttagtttgaatttactgttattcggtgtgcatttctatgtttggtgagcggttttctgtgctcagagtgtgtttattttatgtaatttaatttctttgtgagctcctgtttagcaggtcgtcccttcagcaaggacacaaaaagattttaattttattaaaaaaaaaaaaaaaaaagaccgggaattcgatatcaagcttatcgacctgcagatcgttcaaacatttggcaataaagtttcttaagattgaatcctgttgccggtcttgcgatgattatcatataatttctgttgaattacgttaagcatgtaataattaacatgtaatgcatgacgttatttatgagatgggtttttatgattagagtcccgcaattatacatttaatacgcgatagaaaacaaaatatagcgcgcaaactaggataaattatcgcgcgcggtgtcatctatgttactagat

SEQ ID NO: 54 - protein, 584 aa, Influenza virus
MKAIIVLLMVVTSNADRICTGITSSNSPHVVKTATQGEVNVTGVIPLTTTPTKSYFANLKGTRTRGKLCPDCLNCTDLDVALGRPMCVGTTPSAKASILHEVRPVTSGCFPIMHDRTKIRQLPNLLRGYENIRLSTQNVIDAEKAPGGPYRLGTSGSCPNATSKIGFFATMAWAVPKDNYKNATNPLTVEVPYICTEGEDQITVWGFHSDNKTQMKSLYGDSNPQKFTSSANGVTTHYVSQIGDFPDQTEDGGLPQSGRIVVDYMMQKPGKTGTIVYQRGVLLPQKVWCASGRSKVIKGSLPLIGEADCLHEKYGGLNKSKPYYTGEHAKAIGNCPIWVKTPLKLANGTKYRPPAKLLKERGFFGAIAGFLEGGWEGMIAGWHGYTSHGAHGVAVAADLKSTQEAINKITKNLNSLSELEVKNLQRLSGAMDELHNEILELDEKVDDLRADTISSQIELAVLLSNEGIINSEDEHLLALERKLKKMLGPSAVDIGNGCFETKHKCNQTCLDRIAAGTFNAGEFSLPTFDSLNITAASLNDDGLDNHTILLYYSTAASSLAVTLMLAIFIVYMVSRDNVSCSICL

SEQ ID NO: 55 - DNA, 56 bp, Artificial Sequence
  primer HAB110(PrL-).r
tccttcccatcctccaccaggaggtctatatttggttccattggcaagcttcaaag

SEQ ID NO: 56 - DNA, 52 bp, Artificial Sequence
  primer HAB110(PrL-).c
atatagacctcctggtggaggatgggaaggaatgattgcaggttggcacgga

SEQ ID NO: 57 - DNA, 3444 bp, Artificial Sequence
  Expression cassette number 1467
gtcaacatggtggagcacgacacacttgtctactccaaaaatatcaaagatacagtctcagaagaccaaagggcaattgagacttttcaacaaagggtaatatccggaaacctcctcggattccattgcccagctatctgtcactttattgtgaagatagtggaaaaggaaggtggctcctacaaatgccatcattgcgataaaggaaaggccatcgttgaagatgcctctgccgacagtggtcccaaagatggacccccacccacgaggagcatcgtggaaaaagaagacgttccaaccacgtcttcaaagcaagtggattgatgtgataacatggtggagcacgacacacttgtctactccaaaaatatcaaagatacagtctcagaagaccaaagggcaattgagacttttcaacaaagggtaatatccggaaacctcctcggattccattgcccagctatctgtcactttattgtgaagatagtggaaaaggaaggtggctcctacaaatgccatcattgcgataaaggaaaggccatcgttgaagatgcctctgccgacagtggtcccaaagatggacccccacccacgaggagcatcgtggaaaaagaagacgttccaaccacgtcttcaaagcaagtggattgatgtgatatctccactgacgtaagggatgacgcacaatcccactatccttcgcaagacccttcctctatataaggaagttcatttcatttggagaggtattaaaatcttaataggttttgataaaagcgaacgtggggaaacccgaaccaaaccttcttctaaactctctctcatctctcttaaagcaaacttctctcttgtctttcttgcgtgagcgatcttcaacgttgtcagatcgtgcttcggcaccagtacaacgttttctttcactgaagcgaaatcaaagatctctttgtggacacgtagtgcggcgccattaaataacgtgtacttgtcctattcttgtcggtgtggtcttgggaaaagaaagcttgctggaggctgctgttcagccccatacattacttgttacgattctgctgactttcggcgggtgcaatatctctacttctgcttgacgaggtattgttgcctgtacttctttcttcttcttcttgctgattggttctataagaaatctagtattttctttgaaacagagttttcccgtggttttcgaacttggagaaagattgttaagcttctgtatattctgcccaaatttgtcgggcccatgaaggcaataattgtactactcatggtagtaacatccaatgcagatcgaatctgcactgggataacatcttcaaactcacctcatgtggtcaaaacagctactcaaggggaggtcaatgtgactggcgtgataccactgacaacaacaccaacaaaatcttattttgcaaatctcaaaggaacaaggaccagagggaaactatgcccggactgtctcaactgtacagatctggatgtggccttgggcaggccaatgtgtgtggggaccacaccttctgctaaagcttcaatactccacgaggtcagacctgttacatccgggtgctttcctataatgcacgacagaacaaaaatcaggcaactacccaatcttctcagaggatatgaaaatatcaggttatcaacccaaaacgttatcgatgcagaaaaagcaccaggaggaccctacagacttggaacctcaggatcttgccctaacgctaccagtaaaatcggattttttgcaacaatggcttgggctgtcccaaaggacaactacaaaaatgcaacgaacccactaacagtagaagtaccatacatttgtacagaaggggaagaccaaattactgtttgggggttccattcagataacaaaacccaaatgaagagcctctatggagactcaaatcctcaaaagttcacctcatctgctaatggagtaaccacacattatgtttctcagattggcgacttcccagatcaaacagaagacggaggactaccacaaagcggcagaattgttgttgattacatgatgcaaaaacctgggaaaacaggaacaattgtctatcaaagaggtgttttgttgcctcaaaaggtgtggtgcgcgagtggcaggagcaaagtaataaaagggtcattgcctttaattggtgaagcagattgccttcatgaaaaatacggtggattaaacaaaagcaagccttactacacaggagaacatgcaaaagccataggaaattgcccaatatgggtaaaaacacctttgaagcttgccaatggaaccaaatatagacctcctggtggaggatgggaaggaatgattgcaggttggcacggatacacatctcacggagcacatggagtggcagtggcggcagaccttaagagtacacaagaagctataaataagataacaaaaaatctcaattctttgagtgagctagaagtaaagaaccttcaaagactaagtggtgccatggatgaactccacaacgaaatactcgagctggatgagaaagtggatgatctcagagctgacactataagctcacaaatagaacttgcagtcttgctttccaacgaaggaataataaacagtgaagacgagcatctattggcacttgagagaaaactaaagaaaatgctgggtccctctgctgtagacataggaaacggatgcttcgaaaccaaacacaaatgcaaccagacctgcttagacaggatagctgctggcacctttaatgcaggagaattttctctccccacttttgattcattgaacattactgctgcatctttaaatgatgatggattggataaccatactatactgctctattactcaactgctgcttctagtttggctgtaacattaatgctagctatttttattgtttatatggtctccagagacaacgtttcatgctccatctgtctataaaggcctattttctttagtttgaatttactgttattcggtgtgcatttctatgtttggtgagcggttttctgtgctcagagtgtgtttattttatgtaatttaatttctttgtgagctcctgtttagcaggtcgtcccttcagcaaggacacaaaaagattttaattttattaaaaaaaaaaaaaaaaaagaccgggaattcgatatcaagcttatcgacctgcagatcgttcaaacatttggcaataaagtttcttaagattgaatcctgttgccggtcttgcgatgattatcatataatttctgttgaattacgttaagcatgtaataattaacatgtaatgcatgacgttatttatgagatgggtttttatgattagagtcccgcaattatacatttaatacgcgatagaaaacaaaatatagcgcgcaaactaggataaattatcgcgcgcggtgtcatctatgttactagat

SEQ ID NO: 58 - protein, 567 aa, Influenza virus
MKAIIVLLMVVTSNADRICTGITSSNSPHVVKTATQGEVNVTGVIPLTTTPTKSYFANLKGTRTRGKLCPDCLNCTDLDVALGRPMCVGTTPSAKASILHEVRPVTSGCFPIMHDRTKIRQLPNLLRGYENIRLSTQNVIDAEKAPGGPYRLGTSGSCPNATSKIGFFATMAWAVPKDNYKNATNPLTVEVPYICTEGEDQITVWGFHSDNKTQMKSLYGDSNPQKFTSSANGVTTHYVSQIGDFPDQTEDGGLPQSGRIVVDYMMQKPGKTGTIVYQRGVLLPQKVWCASGRSKVIKGSLPLIGEADCLHEKYGGLNKSKPYYTGEHAKAIGNCPIWVKTPLKLANGTKYRPPGGGWEGMIAGWHGYTSHGAHGVAVAADLKSTQEAINKITKNLNSLSELEVKNLQRLSGAMDELHNEILELDEKVDDLRADTISSQIELAVLLSNEGIINSEDEHLLALERKLKKMLGPSAVDIGNGCFETKHKCNQTCLDRIAAGTFNAGEFSLPTFDSLNITAASLNDDGLDNHTILLYYSTAASSLAVTLMLAIFIVYMVSRDNVSCSICL

SEQ ID NO: 59 - DNA, 44 bp, Artificial Sequence
  primer IF-HB-M-04.s2+4c
tctcagatcttcgccgatcgaatctgcactgggataacatcgtc

SEQ ID NO: 60 - DNA, 46 bp, Artificial Sequence
  primer IF-HB-M-04.s1-4r
actaaagaaaataggcctttatagacagatggagcaagaaacattg

SEQ ID NO: 61 - DNA, 1713 bp, Artificial Sequence
  nucleotide sequence of synthesized HA B Malaysia
gatcgaatctgcactgggataacatcgtcaaactcaccacatgttgtcaaaactgctactcaaggggaggtcaatgtgactggtgtaataccactgacaacaacacccaccaaatctcattttgcaaatctcaaaggaacagaaaccagagggaaactatgcccaaaatgcctcaactgcacagatctggacgtggccttgggcagaccaaaatgcacggggaacataccctcggcaagagtttcaatactccatgaagtcagacctgttacatctgggtgctttcctataatgcacgacagaacaaaaattagacagctgcctaaacttctcagaggatacgaacatatcaggttatcaactcataacgttatcaatgcagaaaatgcaccaggaggaccctacaaaattggaacctcagggtcttgccctaacgttaccaatggaaacggatttttcgcaacaatggcttgggccgtcccaaaaaacgacaacaacaaaacagcaacaaattcattaacaatagaagtaccatacatttgtacagaaggagaagaccaaattaccgtttgggggttccactctgataacgaaacccaaatggcaaagctctatggggactcaaagccccagaagttcacctcatctgccaacggagtgaccacacattacgtttcacagattggtggcttcccaaatcaaacagaagacggaggactaccacaaagcggtagaattgttgttgattacatggtgcaaaaatctgggaaaacaggaacaattacctatcaaagaggtattttattgcctcaaaaagtgtggtgcgcaagtggcaggagcaaggtaataaaaggatcgttgcctttaattggagaagcagattgcctccacgaaaaatacggtggattaaacaaaagcaagccttactacacaggggaacatgcaaaggccataggaaattgcccaatatgggtgaaaacacccttgaagctggccaatggaaccaaatatagacctcctgcaaaactattaaaggaaaggggtttcttcggagctattgctggtttcttagaaggaggatgggaaggaatgattgcaggttggcacggatacacatcccatggggcacatggagtagcggtggcagcagaccttaagagcactcaagaggccataaacaagataacaaaaaatctcaactctttgagtgagctggaagtaaagaatcttcaaagactaagcggtgccatggatgaactccacaacgaaatactagaactagacgagaaagtggatgatctcagagctgatacaataagctcacaaatagaactcgcagtcctgctttccaatgaaggaataataaacagtgaagatgagcatctcttggcgcttgaaagaaagctgaagaaaatgctgggcccctctgctgtagagatagggaatggatgctttgaaaccaaacacaagtgcaaccagacctgtctcgacagaatagctgctggtacctttgatgcaggagaattttctctccccacttttgattcactgaatattactgctgcatctttaaatgacgatggattggataatcatactatactgctttactactcaactgctgcctccagtttggctgtaacattgatgatagctatctttgttgtttatatggtctccagagacaatgtttcttgctccatctgtctataa

SEQ ID NO: 62 - DNA, 6739 bp, Artificial Sequence
  Construct 194
tggcaggatatattgtggtgtaaacaaattgacgcttagacaacttaataacacattgcggacgtttttaatgtactgaattaacgccgaatcccgggctggtatatttatatgttgtcaaataactcaaaaaccataaaagtttaagttagcaagtgtgtacatttttacttgaacaaaaatattcacctactactgttataaatcattattaaacattagagtaaagaaatatggatgataagaacaagagtagtgatattttgacaacaattttgttgcaacatttgagaaaattttgttgttctctcttttcattggtcaaaaacaatagagagagaaaaaggaagagggagaataaaaacataatgtgagtatgagagagaaagttgtacaaaagttgtaccaaaatagttgtacaaatatcattgaggaatttgacaaaagctacacaaataagggttaattgctgtaaataaataaggatgacgcattagagagatgtaccattagagaatttttggcaagtcattaaaaagaaagaataaattatttttaaaattaaaagttgagtcatttgattaaacatgtgattatttaatgaattgatgaaagagttggattaaagttgtattagtaattagaatttggtgtcaaatttaatttgacatttgatcttttcctatatattgccccatagagtcagttaactcatttttatatttcatagatcaaataagagaaataacggtatattaatccctccaaaaaaaaaaaacggtatatttactaaaaaatctaagccacgtaggaggataacaggatccccgtaggaggataacatccaatccaaccaatcacaacaatcctgatgagataacccactttaagcccacgcatctgtggcacatctacattatctaaatcacacattcttccacacatctgagccacacaaaaaccaatccacatctttatcacccattctataaaaaatcacactttgtgagtctacactttgattcccttcaaacacatacaaagagaagagactaattaattaattaatcatcttgagagaaaatggaacgagctatacaaggaaacgacgctagggaacaagctaacagtgaacgttgggatggaggatcaggaggtaccacttctcccttcaaacttcctgacgaaagtccgagttggactgagtggcggctacataacgatgagacgaattcgaatcaagataatccccttggtttcaaggaaagctggggtttcgggaaagttgtatttaagagatatctcagatacgacaggacggaagcttcactgcacagagtccttggatcttggacgggagattcggttaactatgcagcatctcgatttttcggtttcgaccagatcggatgtacctatagtattcggtttcgaggagttagtatcaccgtttctggagggtcgcgaactcttcagcatctctgtgagatggcaattcggtctaagcaagaactgctacagcttgccccaatcgaagtggaaagtaatgtatcaagaggatgccctgaaggtactcaaaccttcgaaaaagaaagcgagtaagttaaaatgcttcttcgtctcctatttataatatggtttgttattgttaattttgttcttgtagaagagcttaattaatcgttgttgttatgaaatactatttgtatgagatgaactggtgtaatgtaattcatttacataagtggagtcagaatcagaatgtttcctccataactaactagacatgaagacctgccgcgtacaattgtcttatatttgaacaactaaaattgaacatcttttgccacaactttataagtggttaatatagctcaaatatatggtcaagttcaatagattaataatggaaatatcagttatcgaaattcattaacaatcaacttaacgttattaactactaattttatatcatcccctttgataaatgatagtacaccaattaggaaggagcatgctcgcctaggagattgtcgtttcccgccttcagtttgcaagctgctctagccgtgtagccaatacgcaaaccgcctctccccgcgcgttgggaattactagcgcgtgtcgagacgcgttgttgttgtgactccgaggggttgcctcaaactctatcttataaccggcgtggaggcatggaggcaggggtattttggtcattttaatagatagtggaaaatgacgtggaatttacttaaagacgaagtctttgcgacaagggggggcccacgccgaatttaatattaccggcgtggcccccccttatcgcgagtgctttagcacgagcggtccagatttaaagtagaaaatttcccgcccactagggttaaaggtgttcacactataaaagcatatacgatgtgatggtatttggtcgacaagcttgcatgccggtcaacatggtggagcacgacacacttgtctactccaaaaatatcaaagatacagtctcagaagaccaaagggcaattgagacttttcaacaaagggtaatatccggaaacctcctcggattccattgcccagctatctgtcactttattgtgaagatagtggaaaaggaaggtggctcctacaaatgccatcattgcgataaaggaaaggccatcgttgaagatgcctctgccgacagtggtcccaaagatggacccccacccacgaggagcatcgtggaaaaagaagacgttccaaccacgtcttcaaagcaagtggattgatgtgataacatggtggagcacgacacacttgtctactccaaaaatatcaaagatacagtctcagaagaccaaagggcaattgagacttttcaacaaagggtaatatccggaaacctcctcggattccattgcccagctatctgtcactttattgtgaagatagtggaaaaggaaggtggctcctacaaatgccatcattgcgataaaggaaaggccatcgttgaagatgcctctgccgacagtggtcccaaagatggacccccacccacgaggagcatcgtggaaaaagaagacgttccaaccacgtcttcaaagcaagtggattgatgtgatatctccactgacgtaagggatgacgcacaatcccactatccttcgcaagacccttcctctatataaggaagttcatttcatttggagaggtattaaaatcttaataggttttgataaaagcgaacgtggggaaacccgaaccaaaccttcttctaaactctctctcatctctcttaaagcaaacttctctcttgtctttcttgcgtgagcgatcttcaacgttgtcagatcgtgcttcggcaccagtacaacgttttctttcactgaagcgaaatcaaagatctctttgtggacacgtagtgcggcgccattaaataacgtgtacttgtcctattcttgtcggtgtggtcttgggaaaagaaagcttgctggaggctgctgttcagccccatacattacttgttacgattctgctgactttcggcgggtgcaatatctctacttctgcttgacgaggtattgttgcctgtacttctttcttcttcttcttgctgattggttctataagaaatctagtattttctttgaaacagagttttcccgtggttttcgaacttggagaaagattgttaagcttctgtatattctgcccaaatttgtcgggcccatggcgaaaaacgttgcgattttcggcttattgttttctcttcttgtgttggttccttctcagatcttcgccgcggctcctcagccaaaacgacacccccatctgtctatccactggcccctggatctgctgcccaaactaactccatggtgaccctgggatgcctggtcaagggctatttccctgagccagtgacagtgacctggaactctggatccctgtccagcggtgtgcacaccttcccagctgtcctgcagtctgacctctacactctgagcagctcagtgactgtcccctccagcacctggcccagcgagaccgtcacctgcaacgttgcccacccggccagcagcaccaaggtggacaagaaaattgtgcccagggattgtggttgtaagccttgcatatgtacagtcccagaagtatcatctgtcttcatcttccccccaaagcccaaggatgtgctcaccattactctgactcctaaggtcacgtgtgttgtggtagacatcagcaaggatgatcccgaggtccagttcagctggtttgtagatgatgtggaggtgcacacagctcagacgcaaccccgggaggagcagttcaacagcactttccgctcagtcagtgaacttcccatcatgcaccaggactggctcaatggcaaggagcgatcgctcaccatcaccatcaccatcaccatcaccattaaaggcctattttctttagtttgaatttactgttattcggtgtgcatttctatgtttggtgagcggttttctgtgctcagagtgtgtttattttatgtaatttaatttctttgtgagctcctgtttagcaggtcgtcccttcagcaaggacacaaaaagattttaattttattaaaaaaaaaaaaaaaaaagaccgggaattcgatatcaagcttatcgacctgcagatcgttcaaacatttggcaataaagtttcttaagattgaatcctgttgccggtcttgcgatgattatcatataatttctgttgaattacgttaagcatgtaataattaacatgtaatgcatgacgttatttatgagatgggtttttatgattagagtcccgcaattatacatttaatacgcgatagaaaacaaaatatagcgcgcaaactaggataaattatcgcgcgcggtgtcatctatgttactagatctctagagtctcaagcttggcgcgccataaaatgattattttatgaatatatttcattgtgcaagtagatagaaattacatatgttacataacacacgaaataaacaaaaaaagacaatccaaaaacaaacaccccaaaaaaaataatcactttagataaactcgtatgaggagaggcacgttcagtgactcgacgattcccgagcaaaaaaagtctccccgtcacacatatagtgggtgacgcaattatctttaaagtaatccttctgttgacttgtcattgataacatccagtcttcgtcaggattgcaaagaattatagaagggatcccaccttttattttcttcttttttccatatttagggttgacagtgaaatcagactggcaacctattaattgcttccacaatgggacgaacttgaaggggatgtcgtcgatgatattataggtggcgtgttcatcgtagttggtgaaatcgatggtaccgttccaatagttgtgtcgtccgagacttctagcccaggtggtctttccggtacgagttggtccgcagatgtagaggctggggtgtcggattccattccttccattgtcctggttaaatcggccatccattcaaggtcagattgagcttgttggtatgagacaggatgtatgtaagtataagcgtctatgcttacatggtatagatgggtttccctccaggagtgtagatcttcgtggcagcgaagatctgattctgtgaagggcgacacatacggttcaggttgtggagggaataatttgttggctgaatattccagccattgaagttttgttgcccattcatgagggaattcttccttgatcatgtcaagatattcctccttagacgttgcagtctggataatagttctccatcgtgcgtcagatttgcgaggagagaccttatgatctcggaaatctcctctggttttaatatctccgtcctttgatatgtaatcaaggacttgtttagagtttctagctggctggatattagggtgatttccttcaaaatcgaaaaaagaaggatccctaatacaaggttttttatcaagctggagaagagcatgatagtgggtagtgccatcttgatgaagctcagaagcaacaccaaggaagaaaataagaaaaggtgtgagtttctcccagagaaactggaataaatcatctctttgagatgagcacttgggataggtaaggaaaacatatttagattggagtctgaagttcttactagcagaaggcatgttgttgtgactccgaggggttgcctcaaactctatcttataaccggcgtggaggcatggaggcaggggtattttggtcattttaatagatagtggaaaatgacgtggaatttacttaaagacgaagtctttgcgacaagggggggcccacgccgaatttaatattaccggcgtggcccccccttatcgcgagtgctttagcacgagcggtccagatttaaagtagaaaatttcccgcccactagggttaaaggtgttcacactataaaagcatatacgatgtgatggtatttgactagtggcactggccgtcgttttacaacgtcgtgactgggaaaaccctggcgttacccaacttaatcgccttgcagcacatccccctttcgccagctggcgtaatagcgaagaggcccgcaccgatcgcccttcccaacagttgcgcagcctgaatggcgaatgctagagcagcttgagcttggatcagattgtcgtttcccgccttcagtttaaactatcagtgtttgacaggatatattggcgggtaaacctaagagaaaagagcgttta

SEQ ID NO: 63 - DNA, 3525 bp, Artificial Sequence
  Expression cassette number 1631
gtcaacatggtggagcacgacacacttgtctactccaaaaatatcaaagatacagtctcagaagaccaaagggcaattgagacttttcaacaaagggtaatatccggaaacctcctcggattccattgcccagctatctgtcactttattgtgaagatagtggaaaaggaaggtggctcctacaaatgccatcattgcgataaaggaaaggccatcgttgaagatgcctctgccgacagtggtcccaaagatggacccccacccacgaggagcatcgtggaaaaagaagacgttccaaccacgtcttcaaagcaagtggattgatgtgataacatggtggagcacgacacacttgtctactccaaaaatatcaaagatacagtctcagaagaccaaagggcaattgagacttttcaacaaagggtaatatccggaaacctcctcggattccattgcccagctatctgtcactttattgtgaagatagtggaaaaggaaggtggctcctacaaatgccatcattgcgataaaggaaaggccatcgttgaagatgcctctgccgacagtggtcccaaagatggacccccacccacgaggagcatcgtggaaaaagaagacgttccaaccacgtcttcaaagcaagtggattgatgtgatatctccactgacgtaagggatgacgcacaatcccactatccttcgcaagacccttcctctatataaggaagttcatttcatttggagaggtattaaaatcttaataggttttgataaaagcgaacgtggggaaacccgaaccaaaccttcttctaaactctctctcatctctcttaaagcaaacttctctcttgtctttcttgcgtgagcgatcttcaacgttgtcagatcgtgcttcggcaccagtacaacgttttctttcactgaagcgaaatcaaagatctctttgtggacacgtagtgcggcgccattaaataacgtgtacttgtcctattcttgtcggtgtggtcttgggaaaagaaagcttgctggaggctgctgttcagccccatacattacttgttacgattctgctgactttcggcgggtgcaatatctctacttctgcttgacgaggtattgttgcctgtacttctttcttcttcttcttgctgattggttctataagaaatctagtattttctttgaaacagagttttcccgtggttttcgaacttggagaaagattgttaagcttctgtatattctgcccaaatttgtcgggcccatggcgaaaaacgttgcgattttcggcttattgttttctcttcttgtgttggttccttctcagatcttcgccgatcgaatctgcactgggataacatcgtcaaactcaccacatgttgtcaaaactgctactcaaggggaggtcaatgtgactggtgtaataccactgacaacaacacccaccaaatctcattttgcaaatctcaaaggaacagaaaccagagggaaactatgcccaaaatgcctcaactgcacagatctggacgtggccttgggcagaccaaaatgcacggggaacataccctcggcaagagtttcaatactccatgaagtcagacctgttacatctgggtgctttcctataatgcacgacagaacaaaaattagacagctgcctaaacttctcagaggatacgaacatatcaggttatcaactcataacgttatcaatgcagaaaatgcaccaggaggaccctacaaaattggaacctcagggtcttgccctaacgttaccaatggaaacggatttttcgcaacaatggcttgggccgtcccaaaaaacgacaacaacaaaacagcaacaaattcattaacaatagaagtaccatacatttgtacagaaggagaagaccaaattaccgtttgggggttccactctgataacgaaacccaaatggcaaagctctatggggactcaaagccccagaagttcacctcatctgccaacggagtgaccacacattacgtttcacagattggtggcttcccaaatcaaacagaagacggaggactaccacaaagcggtagaattgttgttgattacatggtgcaaaaatctgggaaaacaggaacaattacctatcaaagaggtattttattgcctcaaaaagtgtggtgcgcaagtggcaggagcaaggtaataaaaggatcgttgcctttaattggagaagcagattgcctccacgaaaaatacggtggattaaacaaaagcaagccttactacacaggggaacatgcaaaggccataggaaattgcccaatatgggtgaaaacacccttgaagctggccaatggaaccaaatatagacctcctgcaaaactattaaaggaaaggggtttcttcggagctattgctggtttcttagaaggaggatgggaaggaatgattgcaggttggcacggatacacatcccatggggcacatggagtagcggtggcagcagaccttaagagcactcaagaggccataaacaagataacaaaaaatctcaactctttgagtgagctggaagtaaagaatcttcaaagactaagcggtgccatggatgaactccacaacgaaatactagaactagacgagaaagtggatgatctcagagctgatacaataagctcacaaatagaactcgcagtcctgctttccaatgaaggaataataaacagtgaagatgagcatctcttggcgcttgaaagaaagctgaagaaaatgctgggcccctctgctgtagagatagggaatggatgctttgaaaccaaacacaagtgcaaccagacctgtctcgacagaatagctgctggtacctttgatgcaggagaattttctctccccacttttgattcactgaatattactgctgcatctttaaatgacgatggattggataatcatactatactgctttactactcaactgctgcctccagtttggctgtaacattgatgatagctatctttgttgtttatatggtctccagagacaatgtttcttgctccatctgtctataaaggcctattttctttagtttgaatttactgttattcggtgtgcatttctatgtttggtgagcggttttctgtgctcagagtgtgtttattttatgtaatttaatttctttgtgagctcctgtttagcaggtcgtcccttcagcaaggacacaaaaagattttaattttattaaaaaaaaaaaaaaaaaagaccgggaattcgatatcaagcttatcgacctgcagatcgttcaaacatttggcaataaagtttcttaagattgaatcctgttgccggtcttgcgatgattatcatataatttctgttgaattacgttaagcatgtaataattaacatgtaatgcatgacgttatttatgagatgggtttttatgattagagtcccgcaattatacatttaatacgcgatagaaaacaaaatatagcgcgcaaactaggataaattatcgcgcgcggtgtcatctatgttactagat

SEQ ID NO: 64 - protein, 594 aa, Influenza virus
MAKNVAIFGLLFSLLVLVPSQIFADRICTGITSSNSPHVVKTATQGEVNVTGVIPLTTTPTKSHFANLKGTETRGKLCPKCLNCTDLDVALGRPKCTGNIPSARVSILHEVRPVTSGCFPIMHDRTKIRQLPKLLRGYEHIRLSTHNVINAENAPGGPYKIGTSGSCPNVTNGNGFFATMAWAVPKNDNNKTATNSLTIEVPYICTEGEDQITVWGFHSDNETQMAKLYGDSKPQKFTSSANGVTTHYVSQIGGFPNQTEDGGLPQSGRIVVDYMVQKSGKTGTITYQRGILLPQKVWCASGRSKVIKGSLPLIGEADCLHEKYGGLNKSKPYYTGEHAKAIGNCPIWVKTPLKLANGTKYRPPAKLLKERGFFGAIAGFLEGGWEGMIAGWHGYTSHGAHGVAVAADLKSTQEAINKITKNLNSLSELEVKNLQRLSGAMDELHNEILELDEKVDDLRADTISSQIELAVLLSNEGIINSEDEHLLALERKLKKMLGPSAVEIGNGCFETKHKCNQTCLDRIAAGTFDAGEFSLPTFDSLNITAASLNDDGLDNHTILLYYSTAASSLAVTLMIAIFVVYMVSRDNVSCSICL